European Patent Application EP 4 269 603 A1, published November 1, 2023. Title: TARGETED DNA INTEGRATION WITH LENTIVIRAL VECTORS AND USES THEREOF. Applicant: UNIVERSITAT POMPEU FABRA GÜELL CARGOL Marc SÁNCHEZ-MEJÍAS GARCIA Avencia IVANČIĆ Dimitrije. The sequence listing filed with the application follows.

SEQUENCE LISTING (78 sequences)

SEQ ID NO: 1 - protein, 288 aa, Human immunodeficiency virus 1
  HIV-1 Integrase (IN)
FLDGIDKAQEEHEKYHSNWRAMASDFNLPPVVAKEIVASCDKCQLKGEAMHGQVDCSPGIWQLDCTHLEGKVILVAVHVASGYIEAEVIPAETGQETAYFLLKLAGRWPVKTVHTDNGSNFTSTTVKAACWWAGIKQEFGIPYNPQSQGVIESMNKELKKIIGQVRDQAEHLKTAVQMAVFIHNFKRKGGIGGYSAGERIVDIIATDIQTKELQKQITKIQNFRVYYRDSRDPVWKGPAKLLWKGEGAVVIQDNSDIKVVPRRKAKIIRDYGKQMAGDDCVASRQDED

SEQ ID NO: 2 - protein, 288 aa, Human immunodeficiency virus 1
  HIV-1 IN E10K/E13K
FLDGIDKAQKEHKKYHSNWRAMASDFNLPPVVAKEIVASCDKCQLKGEAMHGQVDCSPGIWQLDCTHLEGKVILVAVHVASGYIEAEVIPAETGQETAYFLLKLAGRWPVKTVHTDNGSNFTSTTVKAACWWAGIKQEFGIPYNPQSQGVIESMNKELKKIIGQVRDQAEHLKTAVQMAVFIHNFKRKGGIGGYSAGERIVDIIATDIQTKELQKQITKIQNFRVYYRDSRDPVWKGPAKLLWKGEGAVVIQDNSDIKVVPRRKAKIIRDYGKQMAGDDCVASRQDED

SEQ ID NO: 3 - protein, 288 aa, Human immunodeficiency virus 1
  HIV-1 IN D64V
FLDGIDKAQEEHEKYHSNWRAMASDFNLPPVVAKEIVASCDKCQLKGEAMHGQVDCSPGIWQLVCTHLEGKVILVAVHVASGYIEAEVIPAETGQETAYFLLKLAGRWPVKTVHTDNGSNFTSTTVKAACWWAGIKQEFGIPYNPQSQGVIESMNKELKKIIGQVRDQAEHLKTAVQMAVFIHNFKRKGGIGGYSAGERIVDIIATDIQTKELQKQITKIQNFRVYYRDSRDPVWKGPAKLLWKGEGAVVIQDNSDIKVVPRRKAKIIRDYGKQMAGDDCVASRQDED

SEQ ID NO: 4 - protein, 288 aa, Human immunodeficiency virus 1
  HIV-1 IN D116N
FLDGIDKAQEEHEKYHSNWRAMASDFNLPPVVAKEIVASCDKCQLKGEAMHGQVDCSPGIWQLDCTHLEGKVILVAVHVASGYIEAEVIPAETGQETAYFLLKLAGRWPVKTVHTNNGSNFTSTTVKAACWWAGIKQEFGIPYNPQSQGVIESMNKELKKIIGQVRDQAEHLKTAVQMAVFIHNFKRKGGIGGYSAGERIVDIIATDIQTKELQKQITKIQNFRVYYRDSRDPVWKGPAKLLWKGEGAVVIQDNSDIKVVPRRKAKIIRDYGKQMAGDDCVASRQDED

SEQ ID NO: 5 - protein, 288 aa, Human immunodeficiency virus 1
  HIV-1 IN S119G
FLDGIDKAQEEHEKYHSNWRAMASDFNLPPVVAKEIVASCDKCQLKGEAMHGQVDCSPGIWQLDCTHLEGKVILVAVHVASGYIEAEVIPAETGQETAYFLLKLAGRWPVKTVHTDNGGNFTSTTVKAACWWAGIKQEFGIPYNPQSQGVIESMNKELKKIIGQVRDQAEHLKTAVQMAVFIHNFKRKGGIGGYSAGERIVDIIATDIQTKELQKQITKIQNFRVYYRDSRDPVWKGPAKLLWKGEGAVVIQDNSDIKVVPRRKAKIIRDYGKQMAGDDCVASRQDED

SEQ ID NO: 6 - protein, 288 aa, Human immunodeficiency virus 1
  HIV-1 IN E152V
FLDGIDKAQEEHEKYHSNWRAMASDFNLPPVVAKEIVASCDKCQLKGEAMHGQVDCSPGIWQLDCTHLEGKVILVAVHVASGYIEAEVIPAETGQETAYFLLKLAGRWPVKTVHTDNGSNFTSTTVKAACWWAGIKQEFGIPYNPQSQGVIVSMNKELKKIIGQVRDQAEHLKTAVQMAVFIHNFKRKGGIGGYSAGERIVDIIATDIQTKELQKQITKIQNFRVYYRDSRDPVWKGPAKLLWKGEGAVVIQDNSDIKVVPRRKAKIIRDYGKQMAGDDCVASRQDED

SEQ ID NO: 7 - protein, 288 aa, Human immunodeficiency virus 1
  HIV-1 IN D167H
FLDGIDKAQEEHEKYHSNWRAMASDFNLPPVVAKEIVASCDKCQLKGEAMHGQVDCSPGIWQLDCTHLEGKVILVAVHVASGYIEAEVIPAETGQETAYFLLKLAGRWPVKTVHTDNGSNFTSTTVKAACWWAGIKQEFGIPYNPQSQGVIESMNKELKKIIGQVRHQAEHLKTAVQMAVFIHNFKRKGGIGGYSAGERIVDIIATDIQTKELQKQITKIQNFRVYYRDSRDPVWKGPAKLLWKGEGAVVIQDNSDIKVVPRRKAKIIRDYGKQMAGDDCVASRQDED

SEQ ID NO: 8 - protein, 288 aa, Human immunodeficiency virus 1
  HIV-1 IN K186Q
FLDGIDKAQEEHEKYHSNWRAMASDFNLPPVVAKEIVASCDKCQLKGEAMHGQVDCSPGIWQLDCTHLEGKVILVAVHVASGYIEAEVIPAETGQETAYFLLKLAGRWPVKTVHTDNGSNFTSTTVKAACWWAGIKQEFGIPYNPQSQGVIESMNKELKKIIGQVRDQAEHLKTAVQMAVFIHNFQRKGGIGGYSAGERIVDIIATDIQTKELQKQITKIQNFRVYYRDSRDPVWKGPAKLLWKGEGAVVIQDNSDIKVVPRRKAKIIRDYGKQMAGDDCVASRQDED

SEQ ID NO: 9 - protein, 288 aa, Human immunodeficiency virus 1
  HIV-1 IN R231G
FLDGIDKAQEEHEKYHSNWRAMASDFNLPPVVAKEIVASCDKCQLKGEAMHGQVDCSPGIWQLDCTHLEGKVILVAVHVASGYIEAEVIPAETGQETAYFLLKLAGRWPVKTVHTDNGSNFTSTTVKAACWWAGIKQEFGIPYNPQSQGVIESMNKELKKIIGQVRDQAEHLKTAVQMAVFIHNFKRKGGIGGYSAGERIVDIIATDIQTKELQKQITKIQNFRVYYRDSGDPVWKGPAKLLWKGEGAVVIQDNSDIKVVPRRKAKIIRDYGKQMAGDDCVASRQDED

SEQ ID NO: 10 - protein, 594 aa, Artificial Sequence
  Unmodified Hyperactive Piggybac
MGSSLDDEHILSALLQSDDELVGEDSDSEVSDHVSEDDVQSDTEEAFIDEVHEVQPTSSGSEILDEQNVIEQPGSSLASNRILTLPQRTIRGKNKHCWSTSKPTRRSRVSALNIVRSQRGPTRMCRNIYDPLLCFKLFFTDEIISEIVKWTNAEISLKRRESMTSATFRDTNEDEIYAFFGILVMTAVRKDNHMSTDDLFDRSLSMVYVSVMSRDRFDFLIRCLRMDDKSIRPTLRENDVFTPVRKIWDLFIHQCIQNYTPGAHLTIDEQLLGFRGRCPFRVYIPNKPSKYGIKILMMCDSGTKYMINGMPYLGRGTQTNGVPLGEYYVKELSKPVHGSCRNITCDNWFTSIPLAKNLLQEPYKLTIVGTVRSNKREIPEVLKNSRSRPVGTSMFCFDGPLTLVSYKPKPAKMVYLLSSCDEDASINESTGKPQMVMYYNQTKGGVDTLDQMCSVMTCSRKTNRWPMALLYGMINIACINSFIIYSHNVSSKGEKVQSRKKFMRNLYMGLTSSFMRKRLEAPTLKRYLRDNISNILPKEVPGTSDDSTEEPVMKKRTYCTYCPSKIRRKASASCKKCKKVICREHNIDMCQSCF

SEQ ID NO: 11 - protein, 594 aa, Artificial Sequence
  Modified Hyperactive Piggybac D450N/R372A/K375A
MGSSLDDEHILSALLQSDDELVGEDSDSEVSDHVSEDDVQSDTEEAFIDEVHEVQPTSSGSEILDEQNVIEQPGSSLASNRILTLPQRTIRGKNKHCWSTSKPTRRSRVSALNIVRSQRGPTRMCRNIYDPLLCFKLFFTDEIISEIVKWTNAEISLKRRESMTSATFRDTNEDEIYAFFGILVMTAVRKDNHMSTDDLFDRSLSMVYVSVMSRDRFDFLIRCLRMDDKSIRPTLRENDVFTPVRKIWDLFIHQCIQNYTPGAHLTIDEQLLGFRGRCPFRVYIPNKPSKYGIKILMMCDSGTKYMINGMPYLGRGTQTNGVPLGEYYVKELSKPVHGSCRNITCDNWFTSIPLAKNLLQEPYKLTIVGTVASNAREIPEVLKNSRSRPVGTSMFCFDGPLTLVSYKPKPAKMVYLLSSCDEDASINESTGKPQMVMYYNQTKGGVDTLNQMCSVMTCSRKTNRWPMALLYGMINIACINSFIIYSHNVSSKGEKVQSRKKFMRNLYMGLTSSFMRKRLEAPTLKRYLRDNISNILPKEVPGTSDDSTEEPVMKKRTYCTYCPSKIRRKASASCKKCKKVICREHNIDMCQSCF

SEQ ID NO: 12 - protein, 594 aa, Artificial Sequence
  Modified Hyperactive Piggybac S351A/R372A/K375A/R388A/D450N/W465A/S573A/M589V/592G/S594L
MGSSLDDEHILSALLQSDDELVGEDSDSEVSDHVSEDDVQSDTEEAFIDEVHEVQPTSSGSEILDEQNVIEQPGSSLASNRILTLPQRTIRGKNKHCWSTSKPTRRSRVSALNIVRSQRGPTRMCRNIYDPLLCFKLFFTDEIISEIVKWTNAEISLKRRESMTSATFRDTNEDEIYAFFGILVMTAVRKDNHMSTDDLFDRSLSMVYVSVMSRDRFDFLIRCLRMDDKSIRPTLRENDVFTPVRKIWDLFIHQCIQNYTPGAHLTIDEQLLGFRGRCPFRVYIPNKPSKYGIKILMMCDSGTKYMINGMPYLGRGTQTNGVPLGEYYVKELSKPVHGSCRNITCDNWFTAIPLAKNLLQEPYKLTIVGTVASNAREIPEVLKNSRSAPVGTSMFCFDGPLTLVSYKPKPAKMVYLLSSCDEDASINESTGKPQMVMYYNQTKGGVDTLNQMCSVMTCSRKTNRAPMALLYGMINIACINSFIIYSHNVSSKGEKVQSRKKFMRNLYMGLTSSFMRKRLEAPTLKRYLRDNISNILPKEVPGTSDDSTEEPVMKKRTYCTYCPSKIRRKASAACKKCKKVICREHNIDVCQGCL

SEQ ID NO: 13 - protein, 594 aa, Artificial Sequence
  Modified Hyperactive Piggybac R245A/R275A/R277A/R372A/W465A/M589V
MGSSLDDEHILSALLQSDDELVGEDSDSEVSDHVSEDDVQSDTEEAFIDEVHEVQPTSSGSEILDEQNVIEQPGSSLASNRILTLPQRTIRGKNKHCWSTSKPTRRSRVSALNIVRSQRGPTRMCRNIYDPLLCFKLFFTDEIISEIVKWTNAEISLKRRESMTSATFRDTNEDEIYAFFGILVMTAVRKDNHMSTDDLFDRSLSMVYVSVMSRDRFDFLIRCLRMDDKSIRPTLRENDVFTPVAKIWDLFIHQCIQNYTPGAHLTIDEQLLGFAGACPFRVYIPNKPSKYGIKILMMCDSGTKYMINGMPYLGRGTQTNGVPLGEYYVKELSKPVHGSCRNITCDNWFTSIPLAKNLLQEPYKLTIVGTVASNKREIPEVLKNSRSRPVGTSMFCFDGPLTLVSYKPKPAKMVYLLSSCDEDASINESTGKPQMVMYYNQTKGGVDTLDQMCSVMTCSRKTNRAPMALLYGMINIACINSFIIYSHNVSSKGEKVQSRKKFMRNLYMGLTSSFMRKRLEAPTLKRYLRDNISNILPKEVPGTSDDSTEEPVMKKRTYCTYCPSKIRRKASASCKKCKKVICREHNIDVCQSCF

SEQ ID NO: 14 - protein, 594 aa, Artificial Sequence
  Modified Hyperactive Piggybac R275A/325A/R372A/T560A
MGSSLDDEHILSALLQSDDELVGEDSDSEVSDHVSEDDVQSDTEEAFIDEVHEVQPTSSGSEILDEQNVIEQPGSSLASNRILTLPQRTIRGKNKHCWSTSKPTRRSRVSALNIVRSQRGPTRMCRNIYDPLLCFKLFFTDEIISEIVKWTNAEISLKRRESMTSATFRDTNEDEIYAFFGILVMTAVRKDNHMSTDDLFDRSLSMVYVSVMSRDRFDFLIRCLRMDDKSIRPTLRENDVFTPVRKIWDLFIHQCIQNYTPGAHLTIDEQLLGFAGRCPFRVYIPNKPSKYGIKILMMCDSGTKYMINGMPYLGRGTQTNGVPLAEYYVKELSKPVHGSCRNITCDNWFTSIPLAKNLLQEPYKLTIVGTVASNKREIPEVLKNSRSRPVGTSMFCFDGPLTLVSYKPKPAKMVYLLSSCDEDASINESTGKPQMVMYYNQTKGGVDTLDQMCSVMTCSRKTNRWPMALLYGMINIACINSFIIYSHNVSSKGEKVQSRKKFMRNLYMGLTSSFMRKRLEAPTLKRYLRDNISNILPKEVPGTSDDSTEEPVMKKRTYCAYCPSKIRRKASASCKKCKKVICREHNIDMCQSCF

SEQ ID NO: 15 - protein, 594 aa, Artificial Sequence
  Modified Hyperactive Piggybac S351A/R372A/K375A/R388A/ D450N/W465A/S573A/M589V/S594L
MGSSLDDEHILSALLQSDDELVGEDSDSEVSDHVSEDDVQSDTEEAFIDEVHEVQPTSSGSEILDEQNVIEQPGSSLASNRILTLPQRTIRGKNKHCWSTSKPTRRSRVSALNIVRSQRGPTRMCRNIYDPLLCFKLFFTDEIISEIVKWTNAEISLKRRESMTSATFRDTNEDEIYAFFGILVMTAVRKDNHMSTDDLFDRSLSMVYVSVMSRDRFDFLIRCLRMDDKSIRPTLRENDVFTPVRKIWDLFIHQCIQNYTPGAHLTIDEQLLGFRGRCPFRVYIPNKPSKYGIKILMMCDSGTKYMINGMPYLGRGTQTNGVPLGEYYVKELSKPVHGSCRNITCDNWFTAIPLAKNLLQEPYKLTIVGTVASNAREIPEVLKNSRSAPVGTSMFCFDGPLTLVSYKPKPAKMVYLLSSCDEDASINESTGKPQMVMYYNQTKGGVDTLNQMCSVMTCSRKTNRAPMALLYGMINIACINSFIIYSHNVSSKGEKVQSRKKFMRNLYMGLTSSFMRKRLEAPTLKRYLRDNISNILPKEVPGTSDDSTEEPVMKKRTYCTYCPSKIRRKASAACKKCKKVICREHNIDVCQRCL

SEQ ID NO: 16 - protein, 594 aa, Artificial Sequence
  Modified Hyperactive Piggybac R275A/R277A/N347S/K375A/T560A/S573A/M589V/S594L
MGSSLDDEHILSALLQSDDELVGEDSDSEVSDHVSEDDVQSDTEEAFIDEVHEVQPTSSGSEILDEQNVIEQPGSSLASNRILTLPQRTIRGKNKHCWSTSKPTRRSRVSALNIVRSQRGPTRMCRNIYDPLLCFKLFFTDEIISEIVKWTNAEISLKRRESMTSATFRDTNEDEIYAFFGILVMTAVRKDNHMSTDDLFDRSLSMVYVSVMSRDRFDFLIRCLRMDDKSIRPTLRENDVFTPVRKIWDLFIHQCIQNYTPGAHLTIDEQLLGFAGACPFRVYIPNKPSKYGIKILMMCDSGTKYMINGMPYLGRGTQTNGVPLGEYYVKELSKPVHGSCRNITCDSWFTSIPLAKNLLQEPYKLTIVGTVRSNAREIPEVLKNSRSAPVGTSMFCFDGPLTLVSYKPKPAKMVYLLSSCDEDASINESTGKPQMVMYYNQTKGGVDTLNQMCSVMTCSRKTNRAPMALLYGMINIACINSFIIYSHNVSSKGEKVQSRKKFMRNLYMGLTSSFMRKRLEAPTLKRYLRDNISNILPKEVPGTSDDSTEEPVMKKRTYCAYCPSKIRRKASAACKKCKKVICREHNIDVCQSCL

SEQ ID NO: 17 - protein, 594 aa, Artificial Sequence
  Modified Hyperactive Piggybac R245A/R275A/R277A/R372A/W465A
MGSSLDDEHILSALLQSDDELVGEDSDSEVSDHVSEDDVQSDTEEAFIDEVHEVQPTSSGSEILDEQNVIEQPGSSLASNRILTLPQRTIRGKNKHCWSTSKPTRRSRVSALNIVRSQRGPTRMCRNIYDPLLCFKLFFTDEIISEIVKWTNAEISLKRRESMTSATFRDTNEDEIYAFFGILVMTAVRKDNHMSTDDLFDRSLSMVYVSVMSRDRFDFLIRCLRMDDKSIRPTLRENDVFTPVAKIWDLFIHQCIQNYTPGAHLTIDEQLLGFAGACPFRVYIPNKPSKYGIKILMMCDSGTKYMINGMPYLGRGTQTNGVPLGEYYVKELSKPVHGSCRNITCDNWFTSIPLAKNLLQEPYKLTIVGTVASNKREIPEVLKNSRSRPVGTSMFCFDGPLTLVSYKPKPAKMVYLLSSCDEDASINESTGKPQMVMYYNQTKGGVDTLDQMCSVMTCSRKTNRAPMALLYGMINIACINSFIIYSHNVSSKGEKVQSRKKFMRNLYMGLTSSFMRKRLEAPTLKRYLRDNISNILPKEVPGTSDDSTEEPVMKKRTYCTYCPSKIRRKASASCKKCKKVICREHNIDMCQSCF

SEQ ID NO: 18 - protein, 594 aa, Artificial Sequence
  Modified Hyperactive Piggybac R372A/K375A/R388A/D450N/W465A/S573A/M589V/S594L
MGSSLDDEHILSALLQSDDELVGEDSDSEVSDHVSEDDVQSDTEEAFIDEVHEVQPTSSGSEILDEQNVIEQPGSSLASNRILTLPQRTIRGKNKHCWSTSKPTRRSRVSALNIVRSQRGPTRMCRNIYDPLLCFKLFFTDEIISEIVKWTNAEISLKRRESMTSATFRDTNEDEIYAFFGILVMTAVRKDNHMSTDDLFDRSLSMVYVSVMSRDRFDFLIRCLRMDDKSIRPTLRENDVFTPVRKIWDLFIHQCIQNYTPGAHLTIDEQLLGFRGRCPFRVYIPNKPSKYGIKILMMCDSGTKYMINGMPYLGRGTQTNGVPLGEYYVKELSKPVHGSCRNITCDNWFTSIPLAKNLLQEPYKLTIVGTVASNAREIPEVLKNSRSAPVGTSMFCFDGPLTLVSYKPKPAKMVYLLSSCDEDASINESTGKPQMVMYYNQTKGGVDTLNQMCSVMTCSRKTNRAPMALLYGMINIACINSFIIYSHNVSSKGEKVQSRKKFMRNLYMGLTSSFMRKRLEAPTLKRYLRDNISNILPKEVPGTSDDSTEEPVMKKRTYCTYCPSKIRRKASAACKKCKKVICREHNIDVCQRCL

SEQ ID NO: 19 - protein, 594 aa, Artificial Sequence
  Modified hyperactive PiggyBac R275A/N347S/K375A/D450N/S592G
MGSSLDDEHILSALLQSDDELVGEDSDSEVSDHVSEDDVQSDTEEAFIDEVHEVQPTSSGSEILDEQNVIEQPGSSLASNRILTLPQRTIRGKNKHCWSTSKPTRRSRVSALNIVRSQRGPTRMCRNIYDPLLCFKLFFTDEIISEIVKWTNAEISLKRRESMTSATFRDTNEDEIYAFFGILVMTAVRKDNHMSTDDLFDRSLSMVYVSVMSRDRFDFLIRCLRMDDKSIRPTLRENDVFTPVRKIWDLFIHQCIQNYTPGAHLTIDEQLLGFAGRCPFRVYIPNKPSKYGIKILMMCDSGTKYMINGMPYLGRGTQTNGVPLGEYYVKELSKPVHGSCRNITCDSWFTSIPLAKNLLQEPYKLTIVGTVRSNAREIPEVLKNSRSRPVGTSMFCFDGPLTLVSYKPKPAKMVYLLSSCDEDASINESTGKPQMVMYYNQTKGGVDTLNQMCSVMTCSRKTNRWPMALLYGMINIACINSFIIYSHNVSSKGEKVQSRKKFMRNLYMGLTSSFMRKRLEAPTLKRYLRDNISNILPKEVPGTSDDSTEEPVMKKRTYCTYCPSKIRRKASASCKKCKKVICREHNIDMCQGCF

SEQ ID NO: 20 - protein, 594 aa, Artificial Sequence
  Modified hyperactive PiggyBac N347S/D450N/T560A/S573A/F594L
MGSSLDDEHILSALLQSDDELVGEDSDSEVSDHVSEDDVQSDTEEAFIDEVHEVQPTSSGSEILDEQNVIEQPGSSLASNRILTLPQRTIRGKNKHCWSTSKPTRRSRVSALNIVRSQRGPTRMCRNIYDPLLCFKLFFTDEIISEIVKWTNAEISLKRRESMTSATFRDTNEDEIYAFFGILVMTAVRKDNHMSTDDLFDRSLSMVYVSVMSRDRFDFLIRCLRMDDKSIRPTLRENDVFTPVRKIWDLFIHQCIQNYTPGAHLTIDEQLLGFRGRCPFRVYIPNKPSKYGIKILMMCDSGTKYMINGMPYLGRGTQTNGVPLGEYYVKELSKPVHGSCRNITCDSWFTSIPLAKNLLQEPYKLTIVGTVRSNKREIPEVLKNSRSRPVGTSMFCFDGPLTLVSYKPKPAKMVYLLSSCDEDASINESTGKPQMVMYYNQTKGGVDTLNQMCSVMTCSRKTNRWPMALLYGMINIACINSFIIYSHNVSSKGEKVQSRKKFMRNLYMGLTSSFMRKRLEAPTLKRYLRDNISNILPKEVPGTSDDSTEEPVMKKRTYCAYCPSKIRRKASAACKKCKKVICREHNIDMCQSCL

SEQ ID NO: 21 - protein, 594 aa, Artificial Sequence
  Modified hyperactive PiggyBac N347A/D450N
MGSSLDDEHILSALLQSDDELVGEDSDSEVSDHVSEDDVQSDTEEAFIDEVHEVQPTSSGSEILDEQNVIEQPGSSLASNRILTLPQRTIRGKNKHCWSTSKPTRRSRVSALNIVRSQRGPTRMCRNIYDPLLCFKLFFTDEIISEIVKWTNAEISLKRRESMTSATFRDTNEDEIYAFFGILVMTAVRKDNHMSTDDLFDRSLSMVYVSVMSRDRFDFLIRCLRMDDKSIRPTLRENDVFTPVRKIWDLFIHQCIQNYTPGAHLTIDEQLLGFRGRCPFRVYIPNKPSKYGIKILMMCDSGTKYMINGMPYLGRGTQTNGVPLGEYYVKELSKPVHGSCRNITCDAWFTSIPLAKNLLQEPYKLTIVGTVRSNKREIPEVLKNSRSRPVGTSMFCFDGPLTLVSYKPKPAKMVYLLSSCDEDASINESTGKPQMVMYYNQTKGGVDTLNQMCSVMTCSRKTNRWPMALLYGMINIACINSFIIYSHNVSSKGEKVQSRKKFMRNLYMGLTSSFMRKRLEAPTLKRYLRDNISNILPKEVPGTSDDSTEEPVMKKRTYCTYCPSKIRRKASASCKKCKKVICREHNIDMCQSCF

SEQ ID NO: 22 - protein, 594 aa, Artificial Sequence
  Modified hyperactive PiggyBac R275A/N347S/R372A/D450N/T560A/F594L
MGSSLDDEHILSALLQSDDELVGEDSDSEVSDHVSEDDVQSDTEEAFIDEVHEVQPTSSGSEILDEQNVIEQPGSSLASNRILTLPQRTIRGKNKHCWSTSKPTRRSRVSALNIVRSQRGPTRMCRNIYDPLLCFKLFFTDEIISEIVKWTNAEISLKRRESMTSATFRDTNEDEIYAFFGILVMTAVRKDNHMSTDDLFDRSLSMVYVSVMSRDRFDFLIRCLRMDDKSIRPTLRENDVFTPVRKIWDLFIHQCIQNYTPGAHLTIDEQLLGFAGRCPFRVYIPNKPSKYGIKILMMCDSGTKYMINGMPYLGRGTQTNGVPLGEYYVKELSKPVHGSCRNITCDSWFTSIPLAKNLLQEPYKLTIVGTVASNKREIPEVLKNSRSRPVGTSMFCFDGPLTLVSYKPKPAKMVYLLSSCDEDASINESTGKPQMVMYYNQTKGGVDTLNQMCSVMTCSRKTNRWPMALLYGMINIACINSFIIYSHNVSSKGEKVQSRKKFMRNLYMGLTSSFMRKRLEAPTLKRYLRDNISNILPKEVPGTSDDSTEEPVMKKRTYCAYCPSKIRRKASASCKKCKKVICREHNIDMCQSCL

SEQ ID NO: 23 - protein, 594 aa, Artificial Sequence
  Modified hyperactive PiggyBac R202K/R275A/N347S/R372A/D450N/T560A/F594L
MGSSLDDEHILSALLQSDDELVGEDSDSEVSDHVSEDDVQSDTEEAFIDEVHEVQPTSSGSEILDEQNVIEQPGSSLASNRILTLPQRTIRGKNKHCWSTSKPTRRSRVSALNIVRSQRGPTRMCRNIYDPLLCFKLFFTDEIISEIVKWTNAEISLKRRESMTSATFRDTNEDEIYAFFGILVMTAVRKDNHMSTDDLFDKSLSMVYVSVMSRDRFDFLIRCLRMDDKSIRPTLRENDVFTPVRKIWDLFIHQCIQNYTPGAHLTIDEQLLGFAGRCPFRVYIPNKPSKYGIKILMMCDSGTKYMINGMPYLGRGTQTNGVPLGEYYVKELSKPVHGSCRNITCDSWFTSIPLAKNLLQEPYKLTIVGTVASNKREIPEVLKNSRSRPVGTSMFCFDGPLTLVSYKPKPAKMVYLLSSCDEDASINESTGKPQMVMYYNQTKGGVDTLNQMCSVMTCSRKTNRWPMALLYGMINIACINSFIIYSHNVSSKGEKVQSRKKFMRNLYMGLTSSFMRKRLEAPTLKRYLRDNISNILPKEVPGTSDDSTEEPVMKKRTYCAYCPSKIRRKASASCKKCKKVICREHNIDMCQSCL

SEQ ID NO: 24 - protein, 594 aa, Artificial Sequence
  Modified hyperactive PiggyBac R275A/R277A/N347S/R372A/D450N/T560A/S564P/F594L
MGSSLDDEHILSALLQSDDELVGEDSDSEVSDHVSEDDVQSDTEEAFIDEVHEVQPTSSGSEILDEQNVIEQPGSSLASNRILTLPQRTIRGKNKHCWSTSKPTRRSRVSALNIVRSQRGPTRMCRNIYDPLLCFKLFFTDEIISEIVKWTNAEISLKRRESMTSATFRDTNEDEIYAFFGILVMTAVRKDNHMSTDDLFDRSLSMVYVSVMSRDRFDFLIRCLRMDDKSIRPTLRENDVFTPVRKIWDLFIHQCIQNYTPGAHLTIDEQLLGFAGACPFRVYIPNKPSKYGIKILMMCDSGTKYMINGMPYLGRGTQTNGVPLGEYYVKELSKPVHGSCRNITCDSWFTSIPLAKNLLQEPYKLTIVGTVASNKREIPEVLKNSRSRPVGTSMFCFDGPLTLVSYKPKPAKMVYLLSSCDEDASINESTGKPQMVMYYNQTKGGVDTLNQMCSVMTCSRKTNRWPMALLYGMINIACINSFIIYSHNVSSKGEKVQSRKKFMRNLYMGLTSSFMRKRLEAPTLKRYLRDNISNILPKEVPGTSDDSTEEPVMKKRTYCAYCPPKIRRKASASCKKCKKVICREHNIDMCQSCL

SEQ ID NO: 25 - protein, 594 aa, Artificial Sequence
  Modified Hyperactive Piggybac triple mutant D450N/R372A/K375A/R376A
MGSSLDDEHILSALLQSDDELVGEDSDSEVSDHVSEDDVQSDTEEAFIDEVHEVQPTSSGSEILDEQNVIEQPGSSLASNRILTLPQRTIRGKNKHCWSTSKPTRRSRVSALNIVRSQRGPTRMCRNIYDPLLCFKLFFTDEIISEIVKWTNAEISLKRRESMTSATFRDTNEDEIYAFFGILVMTAVRKDNHMSTDDLFDRSLSMVYVSVMSRDRFDFLIRCLRMDDKSIRPTLRENDVFTPVRKIWDLFIHQCIQNYTPGAHLTIDEQLLGFRGRCPFRVYIPNKPSKYGIKILMMCDSGTKYMINGMPYLGRGTQTNGVPLGEYYVKELSKPVHGSCRNITCDNWFTSIPLAKNLLQEPYKLTIVGTVASNAAEIPEVLKNSRSRPVGTSMFCFDGPLTLVSYKPKPAKMVYLLSSCDEDASINESTGKPQMVMYYNQTKGGVDTLNQMCSVMTCSRKTNRWPMALLYGMINIACINSFIIYSHNVSSKGEKVQSRKKFMRNLYMGLTSSFMRKRLEAPTLKRYLRDNISNILPKEVPGTSDDSTEEPVMKKRTYCTYCPSKIRRKASASCKKCKKVICREHNIDMCQSCF

SEQ ID NO: 26 - protein, 594 aa, Artificial Sequence
  Modified hyperactive PiggyBac R245A/N347S/R372A/D450N/T560A/S564P/S573A/S592G
MGSSLDDEHILSALLQSDDELVGEDSDSEVSDHVSEDDVQSDTEEAFIDEVHEVQPTSSGSEILDEQNVIEQPGSSLASNRILTLPQRTIRGKNKHCWSTSKPTRRSRVSALNIVRSQRGPTRMCRNIYDPLLCFKLFFTDEIISEIVKWTNAEISLKRRESMTSATFRDTNEDEIYAFFGILVMTAVRKDNHMSTDDLFDRSLSMVYVSVMSRDRFDFLIRCLRMDDKSIRPTLRENDVFTPVAKIWDLFIHQCIQNYTPGAHLTIDEQLLGFRGRCPFRVYIPNKPSKYGIKILMMCDSGTKYMINGMPYLGRGTQTNGVPLGEYYVKELSKPVHGSCRNITCDSWFTSIPLAKNLLQEPYKLTIVGTVASNKREIPEVLKNSRSRPVGTSMFCFDGPLTLVSYKPKPAKMVYLLSSCDEDASINESTGKPQMVMYYNQTKGGVDTLNQMCSVMTCSRKTNRWPMALLYGMINIACINSFIIYSHNVSSKGEKVQSRKKFMRNLYMGLTSSFMRKRLEAPTLKRYLRDNISNILPKEVPGTSDDSTEEPVMKKRTYCAYCPPKIRRKASAACKKCKKVICREHNIDMCQGCF

SEQ ID NO: 27 - protein, 594 aa, Artificial Sequence
  Modified hyperactive PiggyBac R277A/G325A/N347A/K375A/D450N/T560A/S564P/S573A/S592G/F594L
MGSSLDDEHILSALLQSDDELVGEDSDSEVSDHVSEDDVQSDTEEAFIDEVHEVQPTSSGSEILDEQNVIEQPGSSLASNRILTLPQRTIRGKNKHCWSTSKPTRRSRVSALNIVRSQRGPTRMCRNIYDPLLCFKLFFTDEIISEIVKWTNAEISLKRRESMTSATFRDTNEDEIYAFFGILVMTAVRKDNHMSTDDLFDRSLSMVYVSVMSRDRFDFLIRCLRMDDKSIRPTLRENDVFTPVRKIWDLFIHQCIQNYTPGAHLTIDEQLLGFRGACPFRVYIPNKPSKYGIKILMMCDSGTKYMINGMPYLGRGTQTNGVPLAEYYVKELSKPVHGSCRNITCDAWFTSIPLAKNLLQEPYKLTIVGTVRSNAREIPEVLKNSRSRPVGTSMFCFDGPLTLVSYKPKPAKMVYLLSSCDEDASINESTGKPQMVMYYNQTKGGVDTLNQMCSVMTCSRKTNRWPMALLYGMINIACINSFIIYSHNVSSKGEKVQSRKKFMRNLYMGLTSSFMRKRLEAPTLKRYLRDNISNILPKEVPGTSDDSTEEPVMKKRTYCAYCPPKIRRKASAACKKCKKVICREHNIDMCQGCL

SEQ ID NO: 28 - protein, 594 aa, Artificial Sequence
  Modified hyperactive PiggyBac V34M/R275A/G325A/N347S/S351A/R372A/K375A/D450N/T560A/S564P
MGSSLDDEHILSALLQSDDELVGEDSDSEVSDHMSEDDVQSDTEEAFIDEVHEVQPTSSGSEILDEQNVIEQPGSSLASNRILTLPQRTIRGKNKHCWSTSKPTRRSRVSALNIVRSQRGPTRMCRNIYDPLLCFKLFFTDEIISEIVKWTNAEISLKRRESMTSATFRDTNEDEIYAFFGILVMTAVRKDNHMSTDDLFDRSLSMVYVSVMSRDRFDFLIRCLRMDDKSIRPTLRENDVFTPVRKIWDLFIHQCIQNYTPGAHLTIDEQLLGFAGRCPFRVYIPNKPSKYGIKILMMCDSGTKYMINGMPYLGRGTQTNGVPLAEYYVKELSKPVHGSCRNITCDSWFTAIPLAKNLLQEPYKLTIVGTVASNAREIPEVLKNSRSRPVGTSMFCFDGPLTLVSYKPKPAKMVYLLSSCDEDASINESTGKPQMVMYYNQTKGGVDTLNQMCSVMTCSRKTNRWPMALLYGMINIACINSFIIYSHNVSSKGEKVQSRKKFMRNLYMGLTSSFMRKRLEAPTLKRYLRDNISNILPKEVPGTSDDSTEEPVMKKRTYCAYCPPKIRRKASASCKKCKKVICREHNIDMCQSCF

SEQ ID NO: 29 - protein, 594 aa, Artificial Sequence
  Modified hyperactive PiggyBac G325A/N347S/K375A/D450N/S573A/M589V/S592G
MGSSLDDEHILSALLQSDDELVGEDSDSEVSDHVSEDDVQSDTEEAFIDEVHEVQPTSSGSEILDEQNVIEQPGSSLASNRILTLPQRTIRGKNKHCWSTSKPTRRSRVSALNIVRSQRGPTRMCRNIYDPLLCFKLFFTDEIISEIVKWTNAEISLKRRESMTSATFRDTNEDEIYAFFGILVMTAVRKDNHMSTDDLFDRSLSMVYVSVMSRDRFDFLIRCLRMDDKSIRPTLRENDVFTPVRKIWDLFIHQCIQNYTPGAHLTIDEQLLGFRGRCPFRVYIPNKPSKYGIKILMMCDSGTKYMINGMPYLGRGTQTNGVPLAEYYVKELSKPVHGSCRNITCDSWFTSIPLAKNLLQEPYKLTIVGTVRSNAREIPEVLKNSRSRPVGTSMFCFDGPLTLVSYKPKPAKMVYLLSSCDEDASINESTGKPQMVMYYNQTKGGVDTLNQMCSVMTCSRKTNRWPMALLYGMINIACINSFIIYSHNVSSKGEKVQSRKKFMRNLYMGLTSSFMRKRLEAPTLKRYLRDNISNILPKEVPGTSDDSTEEPVMKKRTYCTYCPSKIRRKASAACKKCKKVICREHNIDVCQGCF

SEQ ID NO: 30 - protein, 594 aa, Artificial Sequence
  Modified hyperactive PiggyBac S230N/R277A/N347S/K375A/D450N
MGSSLDDEHILSALLQSDDELVGEDSDSEVSDHVSEDDVQSDTEEAFIDEVHEVQPTSSGSEILDEQNVIEQPGSSLASNRILTLPQRTIRGKNKHCWSTSKPTRRSRVSALNIVRSQRGPTRMCRNIYDPLLCFKLFFTDEIISEIVKWTNAEISLKRRESMTSATFRDTNEDEIYAFFGILVMTAVRKDNHMSTDDLFDRSLSMVYVSVMSRDRFDFLIRCLRMDDKNIRPTLRENDVFTPVRKIWDLFIHQCIQNYTPGAHLTIDEQLLGFRGACPFRVYIPNKPSKYGIKILMMCDSGTKYMINGMPYLGRGTQTNGVPLGEYYVKELSKPVHGSCRNITCDSWFTSIPLAKNLLQEPYKLTIVGTVRSNKREIPEVLANSRSRPVGTSMFCFDGPLTLVSYKPKPAKMVYLLSSCDEDASINESTGKPQMVMYYNQTKGGVDTLNQMCSVMTCSRKTNRWPMALLYGMINIACINSFIIYSHNVSSKGEKVQSRKKFMRNLYMGLTSSFMRKRLEAPTLKRYLRDNISNILPKEVPGTSDDSTEEPVMKKRTYCTYCPSKIRRKASASCKKCKKVICREHNIDMCQSCF

SEQ ID NO: 31 - protein, 594 aa, Artificial Sequence
  Modified hyperactive PiggyBac T43I/R372A/K375A/A411T/D450N
MGSSLDDEHILSALLQSDDELVGEDSDSEVSDHVSEDDVQSDIEEAFIDEVHEVQPTSSGSEILDEQNVIEQPGSSLASNRILTLPQRTIRGKNKHCWSTSKPTRRSRVSALNIVRSQRGPTRMCRNIYDPLLCFKLFFTDEIISEIVKWTNAEISLKRRESMTSATFRDTNEDEIYAFFGILVMTAVRKDNHMSTDDLFDRSLSMVYVSVMSRDRFDFLIRCLRMDDKSIRPTLRENDVFTPVRKIWDLFIHQCIQNYTPGAHLTIDEQLLGFRGRCPFRVYIPNKPSKYGIKILMMCDSGTKYMINGMPYLGRGTQTNGVPLGEYYVKELSKPVHGSCRNITCDNWFTSIPLAKNLLQEPYKLTIVGTVASNAREIPEVLKNSRSRPVGTSMFCFDGPLTLVSYKPKPTKMVYLLSSCDEDASINESTGKPQMVMYYNQTKGGVDTLNQMCSVMTCSRKTNRWPMALLYGMINIACINSFIIYSHNVSSKGEKVQSRKKFMRNLYMGLTSSFMRKRLEAPTLKRYLRDNISNILPKEVPGTSDDSTEEPVMKKRTYCTYCPSKIRRKASASCKKCKKVICREHNIDMCQSCF

SEQ ID NO: 32 - protein, 594 aa, Artificial Sequence
  Modified hyperactive PiggyBac G325A/N347S/S351A/K375A/D450N/S573A/M589V/S592G
MGSSLDDEHILSALLQSDDELVGEDSDSEVSDHVSEDDVQSDTEEAFIDEVHEVQPTSSGSEILDEQNVIEQPGSSLASNRILTLPQRTIRGKNKHCWSTSKPTRRSRVSALNIVRSQRGPTRMCRNIYDPLLCFKLFFTDEIISEIVKWTNAEISLKRRESMTSATFRDTNEDEIYAFFGILVMTAVRKDNHMSTDDLFDRSLSMVYVSVMSRDRFDFLIRCLRMDDKSIRPTLRENDVFTPVRKIWDLFIHQCIQNYTPGAHLTIDEQLLGFRGRCPFRVYIPNKPSKYGIKILMMCDSGTKYMINGMPYLGRGTQTNGVPLAEYYVKELSKPVHGSCRNITCDSWFTAIPLAKNLLQEPYKLTIVGTVRSNAREIPEVLKNSRSRPVGTSMFCFDGPLTLVSYKPKPAKMVYLLSSCDEDASINESTGKPQMVMYYNQTKGGVDTLNQMCSVMTCSRKTNRWPMALLYGMINIACINSFIIYSHNVSSKGEKVQSRKKFMRNLYMGLTSSFMRKRLEAPTLKRYLRDNISNILPKEVPGTSDDSTEEPVMKKRTYCTYCPSKIRRKASAACKKCKKVICREHNIDVCQGCF

SEQ ID NO: 33 - protein, 594 aa, Artificial Sequence
  Modified hyperactive PiggyBac Y177H/R275A/G325A/K375A/D450N/T560A/S564P/S592G
MGSSLDDEHILSALLQSDDELVGEDSDSEVSDHVSEDDVQSDTEEAFIDEVHEVQPTSSGSEILDEQNVIEQPGSSLASNRILTLPQRTIRGKNKHCWSTSKPTRRSRVSALNIVRSQRGPTRMCRNIYDPLLCFKLFFTDEIISEIVKWTNAEISLKRRESMTSATFRDTNEDEIHAFFGILVMTAVRKDNHMSTDDLFDRSLSMVYVSVMSRDRFDFLIRCLRMDDKSIRPTLRENDVFTPVRKIWDLFIHQCIQNYTPGAHLTIDEQLLGFAGRCPFRVYIPNKPSKYGIKILMMCDSGTKYMINGMPYLGRGTQTNGVPLAEYYVKELSKPVHGSCRNITCDNWFTSIPLAKNLLQEPYKLTIVGTVRSNAREIPEVLKNSRSRPVGTSMFCFDGPLTLVSYKPKPAKMVYLLSSCDEDASINESTGKPQMVMYYNQTKGGVDTLNQMCSVMTCSRKTNRWPMALLYGMINIACINSFIIYSHNVSSKGEKVQSRKKFMRNLYMGLTSSFMRKRLEAPTLKRYLRDNISNILPKEVPGTSDDSTEEPVMKKRTYCAYCPGKIRRKASASCKKCKKVICREHNIDMCQGCF

SEQ ID NO: 34 - protein, 1368 aa, Streptococcus pyogenes [sequence omitted]

SEQ ID NO: 35 - protein, 1069 aa, Staphylococcus aureus
  SaCas9
MAPKKKRKVGIHGVPAAKRNYILGLDIGITSVGYGIIDYETRDVIDAGVRLFKEANVENNEGRRSKRGARRLKRRRRHRIQRVKKLLFDYNLLTDHSELSGINPYEARVKGLSQKLSEEEFSAALLHLAKRRGVHNVNEVEEDTGNELSTKEQISRNSKALEEKYVAELQLERLKKDGEVRGSINRFKTSDYVKEAKQLLKVQKAYHQLDQSFIDTYIDLLETRRTYYEGPGEGSPFGWKDIKEWYEMLMGHCTYFPEELRSVKYAYNADLYNALNDLNNLVITRDENEKLEYYEKFQIIENVFKQKKKPTLKQIAKEILVNEEDIKGYRVTSTGKPEFTNLKVYHDIKDITARKEIIENAELLDQIAKILTIYQSSEDIQEELTNLNSELTQEEIEQISNLKGYTGTHNLSLKAINLILDELWHTNDNQIAIFNRLKLVPKKVDLSQQKEIPTTLVDDFILSPVVKRSFIQSIKVINAIIKKYGLPNDIIIELAREKNSKDAQKMINEMQKRNRQTNERIEEIIRTTGKENAKYLIEKIKLHDMQEGKCLYSLEAIPLEDLLNNPFNYEVDHIIPRSVSFDNSFNNKVLVKQEENSKKGNRTPFQYLSSSDSKISYETFKKHILNLAKGKGRISKTKKEYLLEERDINRFSVQKDFINRNLVDTRYATRGLMNLLRSYFRVNNLDVKVKSINGGFTSFLRRKWKFKKERNKGYKHHAEDALIIANADFIFKEWKKLDKAKKVMENQMFEEKQAESMPEIETEQEYKEIFITPHQIKHIKDFKDYKYSHRVDKKPNRELINDTLYSTRKDDKGNTLIVNNLNGLYDKDNDKLKKLINKSPEKLLMYHHDPQTYQKLKLIMEQYGDEKNPLYKYYEETGNYLTKYSKKDNGPVIKKIKYYGNKLNAHLDITDDYPNSRNKVVKLSLKPYRFDVYLDNGVYKFVTVKNLDVIKKENYYEVNSKCYEEAKKLKKISNQAEFIASFYNNDLIKINGELYRVIGVNNDLLNRIEVNMIDITYREYLENMNDKRPPRIIKTIASKTQSIKKYSTDILGNLYEVKSKKHPQIIKKG

SEQ ID NO: 36 - protein, 1236 aa, Artificial Sequence
  Cpf1
MAPKKKRKVSKLEKFTNCYSLSKTLRFKAIPVGKTQENIDNKRLLVEDEKRAEDYKGVKKLLDRYYLSFINDVLHSIKLKNLNNYISLFRKKTRTEKENKELENLEINLRKEIAKAFKGNEGYKSLFKKDIIETILPEFLDDKDEIALVNSFNGFTTAFTGFFDNRENMFSEEAKSTSIAFRCINENLTRYISNMDIFEKVDAIFDKHEVQEIKEKILNSDYDVEDFFEGEFFNFVLTQEGIDVYNAIIGGFVTESGEKIKGLNEYINLYNQKTKQKLPKFKPLYKQVLSDRESLSFYGEGYTSDEEVLEVFRNTLNKNSEIFSSIKKLEKLFKNFDEYSSAGIFVKNGPAISTISKDIFGEWNVIRDKWNAEYDDIHLKKKAVVTEKYEDDRRKSFKKIGSFSLEQLQEYADADLSVVEKLKEIIIQKVDEIYKVYGSSEKLFDADFVLEKSLKKNDAVVAIMKDLLDSVKSFENYIKAFFGEGKETNRDESFYGDFVLAYDILLKVDHIYDAIRNYVTQKPYSKDKFKLYFQNPQFMGGWDKDKETDYRATILRYGSKYYLAIMDKKYAKCLQKIDKDDVNGNYEKINYKLLPGPNKMLPKVFFSKKWMAYYNPSEDIQKIYKNGTFKKGDMFNLNDCHKLIDFFKDSISRYPKWSNAYDFNFSETEKYKDIAGFYREVEEQGYKVSFESASKKEVDKLVEEGKLYMFQIYNKDFSDKSHGTPNLHTMYFKLLFDENNHGQIRLSGGAELFMRRASLKKEELVVHPANSPIANKNPDNPKKTTTLSYDVYKDKRFSEDQYELHIPIAINKCPKNIFKINTEVRVLLKHDDNPYVIGIDRGERNLLYIVVVDGKGNIVEQYSLNEIINNFNGIRIKTDYHSLLDKKEKERFEARQNWTSIENIKELKAGYISQVVHKICELVEKYDAVIALEDLNSGFKNSRVKVEKQVYQKFEKMLIDKLNYMVDKKSNPCATGGALKGYQITNKFESFKSMSTQNGFIFYIPAWLTSKIDPSTGFVNLLKTKYTSIADSKKFISSFDRIMYVPEEDLFEFALDYKNFSRTDADYIKKWKLYSYGNRIRIFRNPKKNNVFDWEEVCLTSAYKELFNKYGINYQQGDIRALLCEQSDKAFYSSFMALMSLMLQMRNSITGRTDVDFLISPVKNSDGIFYDSRNYEAQENAILPKNADANGAYNIARKVLWAIGQFKKAEDEKLDKVKIAISNKEWLEYAQTSVKH

SEQ ID NO: 37 - protein, 984 aa, Campylobacter jejuni
  CjCas9
MARILAFDIGISSIGWAFSENDELKDCGVRIFTKVENPKTGESLALPRRLARSARKRLARRKARLNHLKHLIANEFKLNYEDYQSFDESLAKAYKGSLISPYELRFRALNELLSKQDFARVILHIAKRRGYDDIKNSDDKEKGAILKAIKQNEEKLANYQSVGEYLYKEYFQKFKENSKEFTNVRNKKESYERCIAQSFLKDELKLIFKKQREFGFSFSKKFEEEVLSVAFYKRALKDFSHLVGNCSFFTDEKRAPKNSPLAFMFVALTRIINLLNNLKNTEGILYTKDDLNALLNEVLKNGTLTYKQTKKLLGLSDDYEFKGEKGTYFIEFKKYKEFIKALGEHNLSQDDLNEIAKDITLIKDEIKLKKALAKYDLNQNQIDSLSKLEFKDHLNISFKALKLVTPLMLEGKKYDEACNELNLKVAINEDKKDFLPAFNETYYKDEVTNPVVLRAIKEYRKVLNALLKKYGKVHKINIELAREVGKNHSQRAKIEKEQNENYKAKKDAELECEKLGLKINSKNILKLRLFKEQKEFCAYSGEKIKISDLQDEKMLEIDHIYPYSRSFDDSYMNKVLVFTKQNQEKLNQTPFEAFGNDSAKWQKIEVLAKNLPTKKQKRILDKNYKDKEQKNFKDRNLNDTRYIARLVLNYTKDYLDFLPLSDDENTKLNDTQKGSKVHVEAKSGMLTSALRHTWGFSAKDRNNHLHHAIDAVIIAYANNSIVKAFSDFKKEQESNSAELYAKKISELDYKNKRKFFEPFSGFRQKVLDKIDEIFVSKPERKKPSGALHEETFRKEEEFYQSYGGKEGVLKALELGKIRKVNGKIVKNGDMFRVDIFKHKKTNKFYAVPIYTMDFALKVLPNKAVARSKKGEIKDWILMDENYEFCFSLYKDSLILIQTKDMQEPEFVYYNAFTSSTVSLIVSKHDNKFETLSKNQKILFKNANEKEVIAKSIGIQNLKVFEKYIVSALGEVTKAEFRQREDFKK

SEQ ID NO: 38 - protein, 1368 aa, Artificial Sequence
  SpCas9 nickase
MDKKYSIGLAIGTNSVGWAVITDEYKVPSKKFKVLGNTDRHSIKKNLIGALLFDSGETAEATRLKRTARRRYTRRKNRICYLQEIFSNEMAKVDDSFFHRLEESFLVEEDKKHERHPIFGNIVDEVAYHEKYPTIYHLRKKLVDSTDKADLRLIYLALAHMIKFRGHFLIEGDLNPDNSDVDKLFIQLVQTYNQLFEENPINASGVDAKAILSARLSKSRRLENLIAQLPGEKKNGLFGNLIALSLGLTPNFKSNFDLAEDAKLQLSKDTYDDDLDNLLAQIGDQYADLFLAAKNLSDAILLSDILRVNTEITKAPLSASMIKRYDEHHQDLTLLKALVRQQLPEKYKEIFFDQSKNGYAGYIDGGASQEEFYKFIKPILEKMDGTEELLVKLNREDLLRKQRTFDNGSIPHQIHLGELHAILRRQEDFYPFLKDNREKIEKILTFRIPYYVGPLARGNSRFAWMTRKSEETITPWNFEEVVDKGASAQSFIERMTNFDKNLPNEKVLPKHSLLYEYFTVYNELTKVKYVTEGMRKPAFLSGEQKKAIVDLLFKTNRKVTVKQLKEDYFKKIECFDSVEISGVEDRFNASLGTYHDLLKIIKDKDFLDNEENEDILEDIVLTLTLFEDREMIEERLKTYAHLFDDKVMKQLKRRRYTGWGRLSRKLINGIRDKQSGKTILDFLKSDGFANRNFMQLIHDDSLTFKEDIQKAQVSGQGDSLHEHIANLAGSPAIKKGILQTVKVVDELVKVMGRHKPENIVIEMARENQTTQKGQKNSRERMKRIEEGIKELGSQILKEHPVENTQLQNEKLYLYYLQNGRDMYVDQELDINRLSDYDVDHIVPQSFLKDDSIDNKVLTRSDKNRGKSDNVPSEEVVKKMKNYWRQLLNAKLITQRKFDNLTKAERGGLSELDKAGFIKRQLVETRQITKHVAQILDSRMNTKYDENDKLIREVKVITLKSKLVSDFRKDFQFYKVREINNYHHAHDAYLNAVVGTALIKKYPKLESEFVYGDYKVYDVRKMIAKSEQEIGKATAKYFFYSNIMNFFKTEITLANGEIRKRPLIETNGETGEIVWDKGRDFATVRKVLSMPQVNIVKKTEVQTGGFSKESILPKRNSDKLIARKKDWDPKKYGGFDSPTVAYSVLVVAKVEKGKSKKLKSVKELLGITIMERSSFEKNPIDFLEAKGYKEVKKDLIIKLPKYSLFELENGRKRMLASAGELQKGNELALPSKYVNFLYLASHYEKLKGSPEDNEQKQLFVEQHKHYLDEIIEQISEFSKRVILADANLDKVLSAYNKHRDKPIREQAENIIHLFTLTNLGAPAAFKYFDTTIDRKRYTSTKEVLDATLIHQSITGLYETRIDLSQLGGD

SEQ ID NO: 39 - protein, 1069 aa, Artificial Sequence
  SaCas9 nickase
MAPKKKRKVGIHGVPAAKRNYILGLAIGITSVGYGIIDYETRDVIDAGVRLFKEANVENNEGRRSKRGARRLKRRRRHRIQRVKKLLFDYNLLTDHSELSGINPYEARVKGLSQKLSEEEFSAALLHLAKRRGVHNVNEVEEDTGNELSTKEQISRNSKALEEKYVAELQLERLKKDGEVRGSINRFKTSDYVKEAKQLLKVQKAYHQLDQSFIDTYIDLLETRRTYYEGPGEGSPFGWKDIKEWYEMLMGHCTYFPEELRSVKYAYNADLYNALNDLNNLVITRDENEKLEYYEKFQIIENVFKQKKKPTLKQIAKEILVNEEDIKGYRVTSTGKPEFTNLKVYHDIKDITARKEIIENAELLDQIAKILTIYQSSEDIQEELTNLNSELTQEEIEQISNLKGYTGTHNLSLKAINLILDELWHTNDNQIAIFNRLKLVPKKVDLSQQKEIPTTLVDDFILSPVVKRSFIQSIKVINAIIKKYGLPNDIIIELAREKNSKDAQKMINEMQKRNRQTNERIEEIIRTTGKENAKYLIEKIKLHDMQEGKCLYSLEAIPLEDLLNNPFNYEVDHIIPRSVSFDNSFNNKVLVKQEENSKKGNRTPFQYLSSSDSKISYETFKKHILNLAKGKGRISKTKKEYLLEERDINRFSVQKDFINRNLVDTRYATRGLMNLLRSYFRVNNLDVKVKSINGGFTSFLRRKWKFKKERNKGYKHHAEDALIIANADFIFKEWKKLDKAKKVMENQMFEEKQAESMPEIETEQEYKEIFITPHQIKHIKDFKDYKYSHRVDKKPNRELINDTLYSTRKDDKGNTLIVNNLNGLYDKDNDKLKKLINKSPEKLLMYHHDPQTYQKLKLIMEQYGDEKNPLYKYYEETGNYLTKYSKKDNGPVIKKIKYYGNKLNAHLDITDDYPNSRNKVVKLSLKPYRFDVYLDNGVYKFVTVKNLDVIKKENYYEVNSKCYEEAKKLKKISNQAEFIASFYNNDLIKINGELYRVIGVNNDLLNRIEVNMIDITYREYLENMNDKRPPRIIKTIASKTQSIKKYSTDILGNLYEVKSKKHPQIIKKG

SEQ ID NO: 40 - protein, 1368 aa, Artificial Sequence [sequence omitted]

SEQ ID NO: 41 - protein, 990 aa, Artificial Sequence
  CasX
MAPKKKRKVSMQEIKRINKIRRRLVKDSNTKKAGKTGPMKTLLVRVMTPDLRERLENLRKKPENIPQPISNTSRANLNKLLTDYTEMKKAILHVYWEEFQKDPVGLMSRVAQPAPKNIDQRKLIPVKDGNERLTSSGFACSQCCQPLYVYKLEQVNDKGKPHTNYFGRCNVSEHERLILLSPHKPEANDELVTYSLGKFGQRALDFYSIHVTRESNHPVKPLEQIGGNSCASGPVGKALSDACMGAVASFLTKYQDIILEHQKVIKKNEKRLANLKDIASANGLAFPKITLPPQPHTKEGIEAYNNVVAQIVIWVNLNLWQKLKIGRDEAKPLQRLKGFPSFPLVERQANEVDWWDMVCNVKKLINEKKEDGKVFWQNLAGYKRQEALLPYLSSEEDRKKGKKFARYQFGDLLLHLEKKHGEDWGKVYDEAWERIDKKVEGLSKHIKLEEERRSEDAQSKAALTDWLRAKASFVIEGLKEADKDEFCRCELKLQKWYGDLRGKPFAIEAENSILDISGFSKQYNCAFIWQKDGVKKLNLYLIINYFKGGKLRFKKIKPEAFEANRFYTVINKKSGEIVPMEVNFNFDDPNLIILPLAFGKRQGREFIWNDLLSLETGSLKLANGRVIEKTLYNRRTRQDEPALFVALTFERREVLDSSNIKPMNLIGIDRGENIPAVIALTDPEGCPLSRFKDSLGNPTHILRIGESYKEKQRTIQAAKEVEQRRAGGYSRKYASKAKNLADDMVRNTARDLLYYAVTQDAMLIFENLSRGFGRQGKRTFMAERQYTRMEDWLTAKLAYEGLPSKTYLSKTLAQYTSKTCSNCGFTITSADYDRVLEKLKKTATGWMTTINGKELKVEGQITYYNRYKRQNVVKDLSVELDRLSEESVNNDISSWTKGRSGEALSLLKKRFSHRPVQEKFVCLNCGFETHADEQAALNIARSWLFLRSQEYKKYQTNKTTGNTDKRAFVETWQSFYRKKLKEVWKPAVTS

SEQ ID NO: 42 - protein, 860 aa, Artificial Sequence
  dead Cas9
MDKKYSIGLAIGTNSVGWAVITDEYKVPSKKFKVLGNTDRHSIKKNLIGALLFDSGETAEATRLKRTARRRYTRRKNRICYLQEIFSNEMAKVDDSFFHRLEESFLVEEDKKHERHPIFGNIVDEVAYHEKYPTIYHLRKKLVDSTDKADLRLIYLALAHMIKFRGHFLIEGDLNPDNSDVDKLFIQLVQTYNQLFEENPINASGVDAKAILSARLSKSRRLENLIAQLPGEKKNGLFGNLIALSLGLTPNFKSNFDLAEDAKLQLSKDTYDDDLDNLLAQIGDQYADLFLAAKNLSDAILLSDILRVNTEITKAPLSASMIKRYDEHHQDLTLLKALVRQQLPEKYKEIFFDQSKNGYAGYIDGGASQEEFYKFIKPILEKMDGTEELLVKLNREDLLRKQRTFDNGSIPHQIHLGELHAILRRQEDFYPFLKDNREKIEKILTFRIPYYVGPLARGNSRFAWMTRKSEETITPWNFEEVVDKGASAQSFIERMTNFDKNLPNEKVLPKHSLLYEYFTVYNELTKVKYVTEGMRKPAFLSGEQKKAIVDLLFKTNRKVTVKQLKEDYFKKIECFDSVEISGVEDRFNASLGTYHDLLKIIKDKDFLDNEENEDILEDIVLTLTLFEDREMIEERLKTYAHLFDDKVMKQLKRRRYTGWGRLSRKLINGIRDKQSGKTILDFLKSDGFANRNFMQLIHDDSLTFKEDIQKAQVSGQGDSLHEHIANLAGSPAIKKGILQTVKVVDELVKVMGRHKPENIVIEMARENQTTQKGQKNSRERMKRIEEGIKELGSQILKEHPVENTQLQNEKLYLYYLQNGRDMYVDQELDINRLSDYDVAAIVPQSFLKDDSIDNKVLTRS

SEQ ID NO: 43 - protein, 416 aa, Artificial Sequence
  TnpB
MIRNKAFVVRLYPNAAQTELINRTLGSARFVYNHFLARRIAAYKESGKGLTYGQTSSELTLLKQAEETSWLSEVDKFALQNSLKNLETAYKNFFRTVKQSGKKVGFPRFRKKRTGESYRTQFTNNNIQIGEGRLKLPKLGWVKTKGQQDIQGKILNVTVRRIHEGHYEASVLCEVEIPYLPAAPKFAAGVDVGIKDFAIVTDGVRFKHEQNPKYYRSTLKRLRKAQQTLSRRKKGSARYGKAKTKLARIHKRIVNKRQDFLHKLTTSLVREYEIIGTEHLKPDNMRKNRRLALSISDAGWGEFIRQLEYKAAWYGRLVSKVSPYFPSSQLCHDCGFKNPEVKNLAVRTWTCPNCGETHDRDENAALNIRREALVAAGISDTLNAHGGYVRPASAGNGLRSENHATLVVSRADPKKK

SEQ ID NO: 44 - DNA, 30 bp, Artificial Sequence
  GGS3x Linker
ggtggatctggcggtggatctggtggcggt

SEQ ID NO: 45 - protein, 10 aa, Artificial Sequence
  GGS3x Linker
GGSGGGSGGG

SEQ ID NO: 46 - DNA, 36 bp, Artificial Sequence
  GGS4x Linker
ggagggagtggtgggtccggtggtagtggcggatcc

SEQ ID NO: 47 - protein, 12 aa, Artificial Sequence
  GGS4x Linker
GGSGGSGGSGGS

SEQ ID NO: 48 - DNA, 45 bp, Artificial Sequence
  GGS5x Linker
ggaggctccggtgggtctggtgggagcggtggtagtggcggatcc

SEQ ID NO: 49 - protein, 15 aa, Artificial Sequence
  GGS5x Linker
GGSGGSGGSGGSGGS

SEQ ID NO: 50 - DNA, 54 bp, Artificial Sequence
  GGS6x Linker
ggaggcagtggtgggagcggtggttccgggggtagtggtggttccgggggatcc

SEQ ID NO: 51 - protein, 16 aa, Artificial Sequence
  GGS6x Linker
GGSGGSGGSGGSGGSG

SEQ ID NO: 52 - DNA, 63 bp, Artificial Sequence
  GGS7x Linker
ggaggttctggaggctccggtgggtccgggggaagtggggggtcaggcggatcaggaggatcc

SEQ ID NO: 53 - protein, 21 aa, Artificial Sequence
  GGS7x Linker
GGSGGSGGSGGSGGSGGSGGS

SEQ ID NO: 54 - DNA, 75 bp, Artificial Sequence
  GGS8x Linker
ggaggtagcggaggttccggagggagcggcgggagtgggggaagcgggggaagtggaggatccgggggaggatcc

SEQ ID NO: 55 - protein, 21 aa, Artificial Sequence
  GGS8x Linker
GGSGGSGGSGGSGGSGGSGGS

SEQ ID NO: 56 - DNA, 48 bp, Artificial Sequence
  XTEN
tccggtagcgaaacaccggggacttcagaatcggccaccccggagtct

SEQ ID NO: 57 - protein, 16 aa, Artificial Sequence
  XTEN
SGSETPGTSESATPES

SEQ ID NO: 58 - DNA, 36 bp, Artificial Sequence
  Linker B
ggaagcgccggtagtgcggctgggtctggcgagttc

SEQ ID NO: 59 - protein, 12 aa, Artificial Sequence
  Linker B
GSAGSAAGSGEF

SEQ ID NO: 60 - DNA, 390 bp, Artificial Sequence
  MCP N55K - DNA
atggcttcaaactttactcagttcgtgctcgtggacaatggtgggacaggggatgtgacagtggctccttctaatttcgctaatggggtggcagagtggatcagctccaactcacggagccaggcctacaaggtgacatgcagcgtcaggcagtctagtgcccagaagagaaagtataccatcaaggtggaggtccccaaagtggctacccagacagtgggcggagtcgaactgcctgtcgccgcttggaggtcctacctgaacatggagctcactatcccaattttcgctaccaattctgactgtgaactcatcgtgaaggcaatgcaggggctcctcaaagacggtaatcctatcccttccgccatcgccgctaactcaggtatctac

SEQ ID NO: 61 - protein, 130 aa, Artificial Sequence
  MCP N55K - Protein
MASNFTQFVLVDNGGTGDVTVAPSNFANGVAEWISSNSRSQAYKVTCSVRQSSAQKRKYTIKVEVPKVATQTVGGVELPVAAWRSYLNMELTIPIFATNSDCELIVKAMQGLLKDGNPIPSAIAANSGIY

SEQ ID NO: 62 - DNA, 162 bp, Artificial Sequence
  gRNA-MS2(tetraloop)-AAVS1-3 spacer (coding DNA plasmid)
ggggccactagggacaggatgttttagagctaggccaacatgaggatcacccatgtctgcagggcctagcaagttaaaataaggctagtccgttatcaacttggccaacatgaggatcacccatgtctgcagggccaagtggcaccgagtcggtgctttttt

SEQ ID NO: 63 - RNA, 162 nt, Artificial Sequence
  gRNA-MS2(tetraloop)-AAVS1-3 spacer
ggggccacuagggacaggauguuuuagagcuaggccaacaugaggaucacccaugucugcagggccuagcaaguuaaaauaaggcuaguccguuaucaacuuggccaacaugaggaucacccaugucugcagggccaaguggcaccgagucggugcuuuuuu

SEQ ID NO: 64 - protein, 853 aa, Artificial Sequence
  MS2M-GAG
MASNFTQFVLVDNGGTGDVTVAPSNFANGVAEWISSNSRSQAYKVTCSVRQSSAQKRKYTIKVEVPKVATQTVGGVELPVAAWRSYLNMELTIPIFATNSDCELIVKAMQGLLKDGNPIPSAIAANSGIYSQNYPIVQSGLRSRAQASNSAVDGTAGPGSMDSGRDFLTLHGLQDDEDLQALLKGSQLLKVKSSSWRRERFYKLQEDCKTIWQESRKVMRTPESQLFSIEDIQEVRMGHRTEGLEKFARDVPEDRCFSIVFKDQRNTLDLIAPSPADAQHWVLGLHKIIHHSGSMDQRQKLQHWIHSCLRKADKNKDNKMSFKELQNFLKELNIQPRAEFTLAARASVLSGGELDRWEKIRLRPGGKKKYKLKHIVWASRELERFAVNPGLLETSEGCRQILGQLQPSLQTGSEELRSLYNTVATLYCVHQRIEIKDTKEALDKIEEEQNKSKKKAQQAAADTGHSSQVSQNYPIVQNIQGQMVHQAISPRTLNAWVKVVEEKAFSPEVIPMFSALSEGATPQDLNTMLNTVGGHQAAMQMLKETINEEAAEWDRVHPVHAGPIAPGQMREPRGSDIAGTTSTLQEQIGWMTNNPPIPVGEIYKRWIILGLNKIVRMYSPTSILDIRQGPKEPFRDYVDRFYKTLRAEQASQEVKNWMTETLLVQNANPDCKTILKALGPAATLEEMMTACQGVGGPGHKARVLAEAMSQVTNTATIMMQRGNFRNQRKMVKCFNCGKEGHTARNCRAPRKKGCWKCGKEGHQMKDCTERQANFLGKIWPSYKGRPGNFLQSRPEPTAPPFLQSRPEPTAPPEESFRSGVETTTPPQKQEPIDKELYPLTSLRSLFGNDPSSQ

SEQ ID NO: 65 - protein, 1734 aa, Artificial Sequence
  MS2M-PH-gagpol-D64V
MASNFTQFVLVDNGGTGDVTVAPSNFANGVAEWISSNSRSQAYKVTCSVRQSSAQKRKYTIKVEVPKVATQTVGGVELPVAAWRSYLNMELTIPIFATNSDCELIVKAMQGLLKDGNPIPSAIAANSGIYSQNYPIVQSGLRSRAQASNSAVDGTAGPGSMDSGRDFLTLHGLQDDEDLQALLKGSQLLKVKSSSWRRERFYKLQEDCKTIWQESRKVMRTPESQLFSIEDIQEVRMGHRTEGLEKFARDVPEDRCFSIVFKDQRNTLDLIAPSPADAQHWVLGLHKIIHHSGSMDQRQKLQHWIHSCLRKADKNKDNKMSFKELQNFLKELNIQPRAEFTLAARASVLSGGELDRWEKIRLRPGGKKKYKLKHIVWASRELERFAVNPGLLETSEGCRQILGQLQPSLQTGSEELRSLYNTVATLYCVHQRIEIKDTKEALDKIEEEQNKSKKKAQQAAADTGHSSQVSQNYPIVQNIQGQMVHQAISPRTLNAWVKVVEEKAFSPEVIPMFSALSEGATPQDLNTMLNTVGGHQAAMQMLKETINEEAAEWDRVHPVHAGPIAPGQMREPRGSDIAGTTSTLQEQIGWMTNNPPIPVGEIYKRWIILGLNKIVRMYSPTSILDIRQGPKEPFRDYVDRFYKTLRAEQASQEVKNWMTETLLVQNANPDCKTILKALGPAATLEEMMTACQGVGGPGHKARVLAEAMSQVTNTATIMMQRGNFRNQRKMVKCFNCGKEGHTARNCRAPRKKGCWKCGKEGHQMKDCTERQANFLGKIWPSYKGRPGNFLQSRPEPTAPPFLQSRPEPTAPPEESFRSGVETTTPPQKQEPIDKELYPLTSLRSLFGNDPSSQRSVASRRPCWTPAPTTPCWRRACPAGGSPRSAASAASSRGSTTRSSRSAATRPSAPCWWDLHLTSSAGTCPRSAAPTSPSAPSRPCPSSPAWTALRSSGPPRRRSRPWWRSAPRWRRRARSARSAPRTPTTPPCSPSRRRTAPSGGSWWTSGSTRGPRTSGRCSWASPTPPARRRRAPCWTWATPTSACPWTRTSGSIPPSPSPASTTRPPASATSTTCCPRAGRAAPPSSRAAQRSWSPSRSRTPTSSISTWTTCTWAATWRSASTGPRSRSGSTCGGAPPPTRSTRRSPHSCGWATSCTPTSGPCSPSCCPRRTAGPTTFRSWWASTGPARSTLASRGSCASCGAQRLPRSPPRRPSWSWPRTGRSRSPCTACTTTPARTSPRSRSRARASGPTRSTRSPSRTRPASTPACAAPTPTTSSPRPCRRSPPRASSGARLLSSSCPSRRRPGRPGGPSTGRPPGFPSGSSTPLPWSCGISWRRSPSWAPRPSTWTAPPTGRPSWARPATPTRAARRWCPPTPPTRRPSCRLSTWPCRTQAWRTSPTASTPWASSRPSPTRARASWTRSSSSSRRRRCTWPGCPPTRASAATSRWTSWAPASGRSCSWTASTRPRTSTRSTTATGGLWLATSTCLPWWLRRSWPAATSASRARPCTARWTAAPASGSWIAPTWRARSWWPCTWPPATSRPRSPPRPARRPPTSCSWPAAGPRPSTPTTAATSPAPPRLPAGGPASSRSSASPTTPSLRAWWRATRSRRSSARGTRPSTRPPCRWPCSSTTSRGRAASAATAPARGSWTSSPPTSRPRSCRSRSPRSRTSGCTTGTAGTLCGRAPPSCCGRARAPWSRTTATSRWCPGGRPRSSGTTASRWPATTAWPPGRTRT

SEQ ID NO: 66 - protein, 1481 aa, Artificial Sequence
  VPR_Cas9
MEQAPEDQGPQREPYNEWTLELLEELKREAVRHFPRPWLHGLGQHIYETYGDTWTGVEAIIRILQRLLFVHFRIGCQHSRIGILRQRRARNGASRSLVSAGIRKVLFLDGIDKMDKKYSIGLDIGTNSVGWAVITDEYKVPSKKFKVLGNTDRHSIKKNLIGALLFDSGETAEATRLKRTARRRYTRRKNRICYLQEIFSNEMAKVDDSFFHRLEESFLVEEDKKHERHPIFGNIVDEVAYHEKYPTIYHLRKKLVDSTDKADLRLIYLALAHMIKFRGHFLIEGDLNPDNSDVDKLFIQLVQTYNQLFEENPINASGVDAKAILSARLSKSRRLENLIAQLPGEKKNGLFGNLIALSLGLTPNFKSNFDLAEDAKLQLSKDTYDDDLDNLLAQIGDQYADLFLAAKNLSDAILLSDILRVNTEITKAPLSASMIKRYDEHHQDLTLLKALVRQQLPEKYKEIFFDQSKNGYAGYIDGGASQEEFYKFIKPILEKMDGTEELLVKLNREDLLRKQRTFDNGSIPHQIHLGELHAILRRQEDFYPFLKDNREKIEKILTFRIPYYVGPLARGNSRFAWMTRKSEETITPWNFEEVVDKGASAQSFIERMTNFDKNLPNEKVLPKHSLLYEYFTVYNELTKVKYVTEGMRKPAFLSGEQKKAIVDLLFKTNRKVTVKQLKEDYFKKIECFDSVEISGVEDRFNASLGTYHDLLKIIKDKDFLDNEENEDILEDIVLTLTLFEDREMIEERLKTYAHLFDDKVMKQLKRRRYTGWGRLSRKLINGIRDKQSGKTILDFLKSDGFANRNFMQLIHDDSLTFKEDIQKAQVSGQGDSLHEHIANLAGSPAIKKGILQTVKVVDELVKVMGRHKPENIVIEMARENQTTQKGQKNSRERMKRIEEGIKELGSQILKEHPVENTQLQNEKLYLYYLQNGRDMYVDQELDINRLSDYDVDHIVPQSFLKDDSIDNKVLTRSDKNRGKSDNVPSEEVVKKMKNYWRQLLNAKLITQRKFDNLTKAERGGLSELDKAGFIKRQLVETRQITKHVAQILDSRMNTKYDENDKLIREVKVITLKSKLVSDFRKDFQFYKVREINNYHHAHDAYLNAVVGTALIKKYPKLESEFVYGDYKVYDVRKMIAKSEQEIGKATAKYFFYSNIMNFFKTEITLANGEIRKRPLIETNGETGEIVWDKGRDFATVRKVLSMPQVNIVKKTEVQTGGFSKESILPKRNSDKLIARKKDWDPKKYGGFDSPTVAYSVLVVAKVEKGKSKKLKSVKELLGITIMERSSFEKNPIDFLEAKGYKEVKKDLIIKLPKYSLFELENGRKRMLASAGELQKGNELALPSKYVNFLYLASHYEKLKGSPEDNEQKQLFVEQHKHYLDEIIEQISEFSKRVILADANLDKVLSAYNKHRDKPIREQAENIIHLFTLTNLGAPAAFKYFDTTIDRKRYTSTKEVLDATLIHQSITGLYETRIDLSQLGGD

SEQ ID NO: 67 - protein, 96 aa, Artificial Sequence
  VPR
MEQAPEDQGPQREPYNEWTLELLEELKREAVRHFPRPWLHGLGQHIYETYGDTWTGVEAIIRILQRLLFVHFRIGCQHSRIGILRQRRARNGASRS

SEQ ID NO: 68 - protein, 288 aa, Artificial Sequence
  HIV-1 IN D164N
FLDGIDKAQEEHEKYHSNWRAMASDFNLPPVVAKEIVASCDKCQLKGEAMHGQVDCSPGIWQLDCTHLEGKVILVAVHVASGYIEAEVIPAETGQETAYFLLKLAGRWPVKTVHTDNGSNFTSTTVKAACWWAGIKQEFGIPYNPQSQGVIESMNKELKKIIGQVRNQAEHLKTAVQMAVFIHNFKRKGGIGGYSAGERIVDIIATDIQTKELQKQITKIQNFRVYYRDSRDPVWKGPAKLLWKGEGAVVIQDNSDIKVVPRRKAKIIRDYGKQMAGDDCVASRQDED

SEQ ID NO: 69 - protein, 1619 aa, Artificial Sequence
  3_E4 pRRE_SpCas9-NLS-link-p75-LEDGF [325â  530] K401E/ K402E/R405E
MMDKKYSIGLDIGTNSVGWAVITDEYKVPSKKFKVLGNTDRHSIKKNLIGALLFDSGETAEATRLKRTARRRYTRRKNRICYLQEIFSNEMAKVDDSFFHRLEESFLVEEDKKHERHPIFGNIVDEVAYHEKYPTIYHLRKKLVDSTDKADLRLIYLALAHMIKFRGHFLIEGDLNPDNSDVDKLFIQLVQTYNQLFEENPINASGVDAKAILSARLSKSRRLENLIAQLPGEKKNGLFGNLIALSLGLTPNFKSNFDLAEDAKLQLSKDTYDDDLDNLLAQIGDQYADLFLAAKNLSDAILLSDILRVNTEITKAPLSASMIKRYDEHHQDLTLLKALVRQQLPEKYKEIFFDQSKNGYAGYIDGGASQEEFYKFIKPILEKMDGTEELLVKLNREDLLRKQRTFDNGSIPHQIHLGELHAILRRQEDFYPFLKDNREKIEKILTFRIPYYVGPLARGNSRFAWMTRKSEETITPWNFEEVVDKGASAQSFIERMTNFDKNLPNEKVLPKHSLLYEYFTVYNELTKVKYVTEGMRKPAFLSGEQKKAIVDLLFKTNRKVTVKQLKEDYFKKIECFDSVEISGVEDRFNASLGTYHDLLKIIKDKDFLDNEENEDILEDIVLTLTLFEDREMIEERLKTYAHLFDDKVMKQLKRRRYTGWGRLSRKLINGIRDKQSGKTILDFLKSDGFANRNFMQLIHDDSLTFKEDIQKAQVSGQGDSLHEHIANLAGSPAIKKGILQTVKVVDELVKVMGRHKPENIVIEMARENQTTQKGQKNSRERMKRIEEGIKELGSQILKEHPVENTQLQNEKLYLYYLQNGRDMYVDQELDINRLSDYDVDHIVPQSFLKDDSIDNKVLTRSDKNRGKSDNVPSEEVVKKMKNYWRQLLNAKLITQRKFDNLTKAERGGLSELDKAGFIKRQLVETRQITKHVAQILDSRMNTKYDENDKLIREVKVITLKSKLVSDFRKDFQFYKVREINNYHHAHDAYLNAVVGTALIKKYPKLESEFVYGDYKVYDVRKMIAKSEQEIGKATAKYFFYSNIMNFFKTEITLANGEIRKRPLIETNGETGEIVWDKGRDFATVRKVLSMPQVNIVKKTEVQTGGFSKESILPKRNSDKLIARKKDWDPKKYGGFDSPTVAYSVLVVAKVEKGKSKKLKSVKELLGITIMERSSFEKNPIDFLEAKGYKEVKKDLIIKLPKYSLFELENGRKRMLASAGELQKGNELALPSKYVNFLYLASHYEKLKGSPEDNEQKQLFVEQHKHYLDEIIEQISEFSKRVILADANLDKVLSAYNKHRDKPIREQAENIIHLFTLTNLGAPAAFKYFDTTIDRKRYTSTKEVLDATLIHQSITGLYETRIDLSQLGGDSRADPKKKRKVGSGGSSGGSSGSETPGTSESATPESSGGSSGGSEQQNKDEGKKPEVKKVEKKRETSMDSRLQRIHAEIKNSLKIDNLDVNRCIEALDELASLQVTMQQAQKHTEMITTLEEIREFKVSQVIMEKSTMLYNKFKNMFLVGEGDSVITQVLNKSLAEQRQHEEANKTKDQGKKGPNKKLEKEQTGSKTLNGGSDAQDGNQPQHNGESNEDSKDNHEASTKKKPSSEERETEISLKDSTLDN

SEQ ID NO: 70 - protein, 1496 aa, Artificial Sequence
  a5_I5 pRRE SpCas9-xten-p75-LEDGF [325â  429]K401E/ K402E/R405E
MMDKKYSIGLDIGTNSVGWAVITDEYKVPSKKFKVLGNTDRHSIKKNLIGALLFDSGETAEATRLKRTARRRYTRRKNRICYLQEIFSNEMAKVDDSFFHRLEESFLVEEDKKHERHPIFGNIVDEVAYHEKYPTIYHLRKKLVDSTDKADLRLIYLALAHMIKFRGHFLIEGDLNPDNSDVDKLFIQLVQTYNQLFEENPINASGVDAKAILSARLSKSRRLENLIAQLPGEKKNGLFGNLIALSLGLTPNFKSNFDLAEDAKLQLSKDTYDDDLDNLLAQIGDQYADLFLAAKNLSDAILLSDILRVNTEITKAPLSASMIKRYDEHHQDLTLLKALVRQQLPEKYKEIFFDQSKNGYAGYIDGGASQEEFYKFIKPILEKMDGTEELLVKLNREDLLRKQRTFDNGSIPHQIHLGELHAILRRQEDFYPFLKDNREKIEKILTFRIPYYVGPLARGNSRFAWMTRKSEETITPWNFEEVVDKGASAQSFIERMTNFDKNLPNEKVLPKHSLLYEYFTVYNELTKVKYVTEGMRKPAFLSGEQKKAIVDLLFKTNRKVTVKQLKEDYFKKIECFDSVEISGVEDRFNASLGTYHDLLKIIKDKDFLDNEENEDILEDIVLTLTLFEDREMIEERLKTYAHLFDDKVMKQLKRRRYTGWGRLSRKLINGIRDKQSGKTILDFLKSDGFANRNFMQLIHDDSLTFKEDIQKAQVSGQGDSLHEHIANLAGSPAIKKGILQTVKVVDELVKVMGRHKPENIVIEMARENQTTQKGQKNSRERMKRIEEGIKELGSQILKEHPVENTQLQNEKLYLYYLQNGRDMYVDQELDINRLSDYDVDHIVPQSFLKDDSIDNKVLTRSDKNRGKSDNVPSEEVVKKMKNYWRQLLNAKLITQRKFDNLTKAERGGLSELDKAGFIKRQLVETRQITKHVAQILDSRMNTKYDENDKLIREVKVITLKSKLVSDFRKDFQFYKVREINNYHHAHDAYLNAVVGTALIKKYPKLESEFVYGDYKVYDVRKMIAKSEQEIGKATAKYFFYSNIMNFFKTEITLANGEIRKRPLIETNGETGEIVWDKGRDFATVRKVLSMPQVNIVKKTEVQTGGFSKESILPKRNSDKLIARKKDWDPKKYGGFDSPTVAYSVLVVAKVEKGKSKKLKSVKELLGITIMERSSFEKNPIDFLEAKGYKEVKKDLIIKLPKYSLFELENGRKRMLASAGELQKGNELALPSKYVNFLYLASHYEKLKGSPEDNEQKQLFVEQHKHYLDEIIEQISEFSKRVILADANLDKVLSAYNKHRDKPIREQAENIIHLFTLTNLGAPAAFKYFDTTIDRKRYTSTKEVLDATLIHQSITGLYETRIDLSQLGGDGSETPGTSESATPESSEQQNKDEGKKPEVKKVEKKRETSMDSRLQRIHAEIKNSLKIDNLDVNRCIEALDELASLQVTMQQAQKHTEMITTLEEIREFKVSQVIMEKSTMLYNKFKNMFLVGEGDSV

SEQ ID NO: 71 - protein, 1591 aa, Artificial Sequence
  a5_I6 pRRE-p75-LEDGF [325â  530]K401E/ K402E/R405E-xten-SpCas9
MSEQQNKDEGKKPEVKKVEKKRETSMDSRLQRIHAEIKNSLKIDNLDVNRCIEALDELASLQVTMQQAQKHTEMITTLEEIREFKVSQVIMEKSTMLYNKFKNMFLVGEGDSVITQVLNKSLAEQRQHEEANKTKDQGKKGPNKKLEKEQTGSKTLNGGSDAQDGNQPQHNGESNEDSKDNHEASTKKKPSSEERETEISLKDSTLDNGSETPGTSESATPESMDKKYSIGLDIGTNSVGWAVITDEYKVPSKKFKVLGNTDRHSIKKNLIGALLFDSGETAEATRLKRTARRRYTRRKNRICYLQEIFSNEMAKVDDSFFHRLEESFLVEEDKKHERHPIFGNIVDEVAYHEKYPTIYHLRKKLVDSTDKADLRLIYLALAHMIKFRGHFLIEGDLNPDNSDVDKLFIQLVQTYNQLFEENPINASGVDAKAILSARLSKSRRLENLIAQLPGEKKNGLFGNLIALSLGLTPNFKSNFDLAEDAKLQLSKDTYDDDLDNLLAQIGDQYADLFLAAKNLSDAILLSDILRVNTEITKAPLSASMIKRYDEHHQDLTLLKALVRQQLPEKYKEIFFDQSKNGYAGYIDGGASQEEFYKFIKPILEKMDGTEELLVKLNREDLLRKQRTFDNGSIPHQIHLGELHAILRRQEDFYPFLKDNREKIEKILTFRIPYYVGPLARGNSRFAWMTRKSEETITPWNFEEVVDKGASAQSFIERMTNFDKNLPNEKVLPKHSLLYEYFTVYNELTKVKYVTEGMRKPAFLSGEQKKAIVDLLFKTNRKVTVKQLKEDYFKKIECFDSVEISGVEDRFNASLGTYHDLLKIIKDKDFLDNEENEDILEDIVLTLTLFEDREMIEERLKTYAHLFDDKVMKQLKRRRYTGWGRLSRKLINGIRDKQSGKTILDFLKSDGFANRNFMQLIHDDSLTFKEDIQKAQVSGQGDSLHEHIANLAGSPAIKKGILQTVKVVDELVKVMGRHKPENIVIEMARENQTTQKGQKNSRERMKRIEEGIKELGSQILKEHPVENTQLQNEKLYLYYLQNGRDMYVDQELDINRLSDYDVDHIVPQSFLKDDSIDNKVLTRSDKNRGKSDNVPSEEVVKKMKNYWRQLLNAKLITQRKFDNLTKAERGGLSELDKAGFIKRQLVETRQITKHVAQILDSRMNTKYDENDKLIREVKVITLKSKLVSDFRKDFQFYKVREINNYHHAHDAYLNAVVGTALIKKYPKLESEFVYGDYKVYDVRKMIAKSEQEIGKATAKYFFYSNIMNFFKTEITLANGEIRKRPLIETNGETGEIVWDKGRDFATVRKVLSMPQVNIVKKTEVQTGGFSKESILPKRNSDKLIARKKDWDPKKYGGFDSPTVAYSVLVVAKVEKGKSKKLKSVKELLGITIMERSSFEKNPIDFLEAKGYKEVKKDLIIKLPKYSLFELENGRKRMLASAGELQKGNELALPSKYVNFLYLASHYEKLKGSPEDNEQKQLFVEQHKHYLDEIIEQISEFSKRVILADANLDKVLSAYNKHRDKPIREQAENIIHLFTLTNLGAPAAFKYFDTTIDRKRYTSTKEVLDATLIHQSITGLYETRIDLSQLGGD

SEQ ID NO: 72 - protein, 1619 aa, Artificial Sequence
  a7_F1 pRRE_SpCas9-shortlink-p75-LEDGF [325â  530]wt
MMDKKYSIGLDIGTNSVGWAVITDEYKVPSKKFKVLGNTDRHSIKKNLIGALLFDSGETAEATRLKRTARRRYTRRKNRICYLQEIFSNEMAKVDDSFFHRLEESFLVEEDKKHERHPIFGNIVDEVAYHEKYPTIYHLRKKLVDSTDKADLRLIYLALAHMIKFRGHFLIEGDLNPDNSDVDKLFIQLVQTYNQLFEENPINASGVDAKAILSARLSKSRRLENLIAQLPGEKKNGLFGNLIALSLGLTPNFKSNFDLAEDAKLQLSKDTYDDDLDNLLAQIGDQYADLFLAAKNLSDAILLSDILRVNTEITKAPLSASMIKRYDEHHQDLTLLKALVRQQLPEKYKEIFFDQSKNGYAGYIDGGASQEEFYKFIKPILEKMDGTEELLVKLNREDLLRKQRTFDNGSIPHQIHLGELHAILRRQEDFYPFLKDNREKIEKILTFRIPYYVGPLARGNSRFAWMTRKSEETITPWNFEEVVDKGASAQSFIERMTNFDKNLPNEKVLPKHSLLYEYFTVYNELTKVKYVTEGMRKPAFLSGEQKKAIVDLLFKTNRKVTVKQLKEDYFKKIECFDSVEISGVEDRFNASLGTYHDLLKIIKDKDFLDNEENEDILEDIVLTLTLFEDREMIEERLKTYAHLFDDKVMKQLKRRRYTGWGRLSRKLINGIRDKQSGKTILDFLKSDGFANRNFMQLIHDDSLTFKEDIQKAQVSGQGDSLHEHIANLAGSPAIKKGILQTVKVVDELVKVMGRHKPENIVIEMARENQTTQKGQKNSRERMKRIEEGIKELGSQILKEHPVENTQLQNEKLYLYYLQNGRDMYVDQELDINRLSDYDVDHIVPQSFLKDDSIDNKVLTRSDKNRGKSDNVPSEEVVKKMKNYWRQLLNAKLITQRKFDNLTKAERGGLSELDKAGFIKRQLVETRQITKHVAQILDSRMNTKYDENDKLIREVKVITLKSKLVSDFRKDFQFYKVREINNYHHAHDAYLNAVVGTALIKKYPKLESEFVYGDYKVYDVRKMIAKSEQEIGKATAKYFFYSNIMNFFKTEITLANGEIRKRPLIETNGETGEIVWDKGRDFATVRKVLSMPQVNIVKKTEVQTGGFSKESILPKRNSDKLIARKKDWDPKKYGGFDSPTVAYSVLVVAKVEKGKSKKLKSVKELLGITIMERSSFEKNPIDFLEAKGYKEVKKDLIIKLPKYSLFELENGRKRMLASAGELQKGNELALPSKYVNFLYLASHYEKLKGSPEDNEQKQLFVEQHKHYLDEIIEQISEFSKRVILADANLDKVLSAYNKHRDKPIREQAENIIHLFTLTNLGAPAAFKYFDTTIDRKRYTSTKEVLDATLIHQSITGLYETRIDLSQLGGDSRADPKKKRKVGSGGSSGGSSGSETPGTSESATPESSGGSSGGSEQQNKDEGKKPEVKKVEKKRETSMDSRLQRIHAEIKNSLKIDNLDVNRCIEALDELASLQVTMQQAQKHTEMITTLKKIRRFKVSQVIMEKSTMLYNKFKNMFLVGEGDSVITQVLNKSLAEQRQHEEANKTKDQGKKGPNKKLEKEQTGSKTLNGGSDAQDGNQPQHNGESNEDSKDNHEASTKKKPSSEERETEISLKDSTLDN

SEQ ID NO: 73 - protein, 1496 aa, Artificial Sequence
  a7_F2 pRRE SpCas9-xten-p75-LEDGF [325â  429]wt
MMDKKYSIGLDIGTNSVGWAVITDEYKVPSKKFKVLGNTDRHSIKKNLIGALLFDSGETAEATRLKRTARRRYTRRKNRICYLQEIFSNEMAKVDDSFFHRLEESFLVEEDKKHERHPIFGNIVDEVAYHEKYPTIYHLRKKLVDSTDKADLRLIYLALAHMIKFRGHFLIEGDLNPDNSDVDKLFIQLVQTYNQLFEENPINASGVDAKAILSARLSKSRRLENLIAQLPGEKKNGLFGNLIALSLGLTPNFKSNFDLAEDAKLQLSKDTYDDDLDNLLAQIGDQYADLFLAAKNLSDAILLSDILRVNTEITKAPLSASMIKRYDEHHQDLTLLKALVRQQLPEKYKEIFFDQSKNGYAGYIDGGASQEEFYKFIKPILEKMDGTEELLVKLNREDLLRKQRTFDNGSIPHQIHLGELHAILRRQEDFYPFLKDNREKIEKILTFRIPYYVGPLARGNSRFAWMTRKSEETITPWNFEEVVDKGASAQSFIERMTNFDKNLPNEKVLPKHSLLYEYFTVYNELTKVKYVTEGMRKPAFLSGEQKKAIVDLLFKTNRKVTVKQLKEDYFKKIECFDSVEISGVEDRFNASLGTYHDLLKIIKDKDFLDNEENEDILEDIVLTLTLFEDREMIEERLKTYAHLFDDKVMKQLKRRRYTGWGRLSRKLINGIRDKQSGKTILDFLKSDGFANRNFMQLIHDDSLTFKEDIQKAQVSGQGDSLHEHIANLAGSPAIKKGILQTVKVVDELVKVMGRHKPENIVIEMARENQTTQKGQKNSRERMKRIEEGIKELGSQILKEHPVENTQLQNEKLYLYYLQNGRDMYVDQELDINRLSDYDVDHIVPQSFLKDDSIDNKVLTRSDKNRGKSDNVPSEEVVKKMKNYWRQLLNAKLITQRKFDNLTKAERGGLSELDKAGFIKRQLVETRQITKHVAQILDSRMNTKYDENDKLIREVKVITLKSKLVSDFRKDFQFYKVREINNYHHAHDAYLNAVVGTALIKKYPKLESEFVYGDYKVYDVRKMIAKSEQEIGKATAKYFFYSNIMNFFKTEITLANGEIRKRPLIETNGETGEIVWDKGRDFATVRKVLSMPQVNIVKKTEVQTGGFSKESILPKRNSDKLIARKKDWDPKKYGGFDSPTVAYSVLVVAKVEKGKSKKLKSVKELLGITIMERSSFEKNPIDFLEAKGYKEVKKDLIIKLPKYSLFELENGRKRMLASAGELQKGNELALPSKYVNFLYLASHYEKLKGSPEDNEQKQLFVEQHKHYLDEIIEQISEFSKRVILADANLDKVLSAYNKHRDKPIREQAENIIHLFTLTNLGAPAAFKYFDTTIDRKRYTSTKEVLDATLIHQSITGLYETRIDLSQLGGDGSETPGTSESATPESSEQQNKDEGKKPEVKKVEKKRETSMDSRLQRIHAEIKNSLKIDNLDVNRCIEALDELASLQVTMQQAQKHTEMITTLKKIRRFKVSQVIMEKSTMLYNKFKNMFLVGEGDSV

SEQ ID NO: 74 - DNA, 7563 bp, Artificial Sequence
  pSICO
acgggccagatatacgcgttgacattgattattgactagttattaatagtaatcaattacggggtcattagttcatagcccatatatggagttccgcgttacataacttacggtaaatggcccgcctggctgaccgcccaacgacccccgcccattgacgtcaataatgacgtatgttcccatagtaacgccaatagggactttccattgacgtcaatgggtggagtatttacggtaaactgcccacttggcagtacatcaagtgtatcatatgccaagtacgccccctattgacgtcaatgacggtaaatggcccgcctggcattatgcccagtacatgaccttatgggactttcctacttggcagtacatctacgtattagtcatcgctattaccatggtgatgcggttttggcagtacatcaatgggcgtggatagcggtttgactcacggggatttccaagtctccaccccattgacgtcaatgggagtttgttttggcaccaaaatcaacgggactttccaaaatgtcgtaacaactccgccccattgacgcaaatgggcggtaggcgtgtacggtgggaggtctatataagcagcgcgttttgcctgtactgggtctctctggttagaccagatctgagcctgggagctctctggctaactagggaacccactgcttaagcctcaataaagcttgccttgagtgcttcaagtagtgtgtgcccgtctgttgtgtgactctggtaactagagatccctcagacccttttagtcagtgtggaaaatctctagcagtggcgcccgaacagggacttgaaagcgaaagggaaaccagaggagctctctcgacgcaggactcggcttgctgaagcgcgcacggcaagaggcgaggggcggcgactggtgagtacgccaaaaattttgactagcggaggctagaaggagagagatgggtgcgagagcgtcagtattaagcgggggagaattagatcgcgatgggaaaaaattcggttaaggccagggggaaagaaaaaatataaattaaaacatatagtatgggcaagcagggagctagaacgattcgcagttaatcctggcctgttagaaacatcagaaggctgtagacaaatactgggacagctacaaccatcccttcagacaggatcagaagaacttagatcattatataatacagtagcaaccctctattgtgtgcatcaaaggatagagataaaagacaccaaggaagctttagacaagatagaggaagagcaaaacaaaagtaagaccaccgcacagcaagcggccggccgctgatcttcagacctggaggaggagatatgagggacaattggagaagtgaattatataaatataaagtagtaaaaattgaaccattaggagtagcacccaccaaggcaaagagaagagtggtgcagagagaaaaaagagcagtgggaataggagctttgttccttgggttcttgggagcagcaggaagcactatgggcgcagcgtcaatgacgctgacggtacaggccagacaattattgtctggtatagtgcagcagcagaacaatttgctgagggctattgaggcgcaacagcatctgttgcaactcacagtctggggcatcaagcagctccaggcaagaatcctggctgtggaaagatacctaaaggatcaacagctcctggggatttggggttgctctggaaaactcatttgcaccactgctgtgccttggaatgctagttggagtaataaatctctggaacagatttggaatcacacgacctggatggagtgggacagagaaattaacaattacacaagcttaatacactccttaattgaagaatcgcaaaaccagcaagaaaagaatgaacaagaattattggaattagataaatgggcaagtttgtggaattggtttaacataacaaattggctgtggtatataaaattattcataatgatagtaggaggcttggtaggtttaagaatagtttttgctgtactttctatagtgaatagagttaggcagggatattcaccattatcgtttcagacccacctcccaaccccgaggggacccgacaggcccgaaggaatagaagaagaaggtggagagagagacagagacagatccattcgattagtgaacggatcggcactgcgtgcgccaattctgcagacaaatggcagtattcatccacaattttaaaagaaaaggggggattggggggtacagtgcaggggaaagaatagtagacataatagcaacagacatacaaactaaagaattacaaaaacaaattacaaaaattcaaaattttcgggtttattacagggacagcagagatccagtttggttagtaccgggcccgctctagagatccgacgcgccatctctaggcccgcgccggccccctcgcacagacttgtgggagaagctcggctactcccctgccccggttaatttgcatataatatttcctagtaactatagaggcttaatgtgcgataaaagacagataatctgttctttttaatactagctacattttacatgataggcttggatttctataagagatacaaatactaaattattattttaaaaaacagcacaaaaggaaactcaccctaactgtaaagtaattataacttcgtatagtataaattatacgaagttataagccttggttttttgaattccgtattaccgccatgcattagttattaatagtaatcaattacggggtcattagttcatagcccatatatggagttccgcgttacataacttacggtaaatggcccgcctggctgaccgcccaacgacccccgcccattgacgtcaataatgacgtatgttcccatagtaacgccaatagggactttccattgacgtcaatgggtggagtatttacggtaaactgcccacttggcagtacatcaagtgtatcatatgccaagtacgccccctattgacgtcaatgacggtaaatggcccgcctggcattatgcccagtacatgaccttatgggactttcctacttggcagtacatctacgtattagtcatcgctattaccatggtgatgcggttttggcagtacatcaatgggcgtggatagcggtttgactcacggggatttccaagtctccaccccattgacgtcaatgggagtttgttttggcaccaaaatcaacgggactttccaaaatgtcgtaacaactccgccccattgacgcaaatgggcggtaggcgtgtacggtgggaggtctatataagcagagctggtttagtgaaccgtcagatccgctagcgctaccggtcgccaccatggtgagcaagggcgaggagctgttcaccggggtggtgcccatcctggtcgagctggacggcgacgtaaacggccacaagttcagcgtgtccggcgagggcgagggcgatgccacctacggcaagctgaccctgaagttcatctgcaccaccggcaagctgcccgtgccctggcccaccctcgtgaccaccctgacctacggcgtgcagtgcttcagccgctaccccgaccacatgaagcagcacgacttcttcaagtccgccatgcccgaaggctacgtccaggagcgcaccatcttcttcaaggacgacggcaactacaagacccgcgccgaggtgaagttcgagggcgacaccctggtgaaccgcatcgagctgaagggcatcgacttcaaggaggacggcaacatcctggggcacaagctggagtacaactacaacagccacaacgtctatatcatggccgacaagcagaagaacggcatcaaggtgaacttcaagatccgccacaacatcgaggacggcagcgtgcagctcgccgaccactaccagcagaacacccccatcggcgacggccccgtgctgctgcccgacaaccactacctgagcacccagtccgccctgagcaaagaccccaacgagaagcgcgatcacatggtcctgctggagttcgtgaccgccgccgggatcactctcggcatggacgagctgtacaagtagcggccgcataacttcgtatagtataaattatacgaagttataagccttgttaacgcgcggtgaccctcgaggtcgacggtatcgataagctcgcttcacgagatcatgtttaagggttccggttccactaggtacaattcgatatcaagcttatcgataatcaacctctggattacaaaatttgtgaaagattgactggtattcttaactatgttgctccttttacgctatgtggatacgctgctttaatgcctttgtatcatgctattgcttcccgtatggctttcattttctcctccttgtataaatcctggttgctgtctctttatgaggagttgtggcccgttgtcaggcaacgtggcgtggtgtgcactgtgtttgctgacgcaacccccactggttggggcattgccaccacctgtcagctcctttccgggactttcgctttccccctccctattgccacggcggaactcatcgccgcctgccttgcccgctgctggacaggggctcggctgttgggcactgacaattccgtggtgttgtcggggaaatcatcgtcctttccttggctgctcgcctgtgttgccacctggattctgcgcgggacgtccttctgctacgtcccttcggccctcaatccagcggaccttccttcccgcggcctgctgccggctctgcggcctcttccgcgtcttcgccttcgccctcagacgagtcggatctccctttgggccgcctccccgcatcgataccgtcgacctcgatcgagacctagaaaaacatggagcaatcacaagtagcaatacagcagctaccaatgctgattgtgcctggctagaagcacaagaggaggaggaggtgggttttccagtcacacctcaggtacctttaagaccaatgacttacaaggcagctgtagatcttagccactttttaaaagaaaaggggggactggaagggctaattcactcccaacgaagacaagatatccttgatctgtggatctaccacacacaaggctacttccctgattggcagaactacacaccagggccagggatcagatatccactgacctttggatggtgctacaagctagtaccagttgagcaagagaaggtagaagaagccaatgaaggagagaacacccgcttgttacaccctgtgagcctgcatgggatggatgacccggagagagaagtattagagtggaggtttgacagccgcctagcatttcatcacatggcccgagagctgcatccggactgtactgggtctctctggttagaccagatctgagcctgggagctctctggctaactagggaacccactgcttaagcctcaataaagcttgccttgagtgcttcaagtagtgtgtgcccgtctgttgtgtgactctggtaactagagatccctcagacccttttagtcagtgtggaaaatctctagcagcatgtgagcaaaaggccagcaaaaggccaggaaccgtaaaaaggccgcgttgctggcgtttttccataggctccgcccccctgacgagcatcacaaaaatcgacgctcaagtcagaggtggcgaaacccgacaggactataaagataccaggcgtttccccctggaagctccctcgtgcgctctcctgttccgaccctgccgcttaccggatacctgtccgcctttctcccttcgggaagcgtggcgctttctcatagctcacgctgtaggtatctcagttcggtgtaggtcgttcgctccaagctgggctgtgtgcacgaaccccccgttcagcccgaccgctgcgccttatccggtaactatcgtcttgagtccaacccggtaagacacgacttatcgccactggcagcagccactggtaacaggattagcagagcgaggtatgtaggcggtgctacagagttcttgaagtggtggcctaactacggctacactagaagaacagtatttggtatctgcgctctgctgaagccagttaccttcggaaaaagagttggtagctcttgatccggcaaacaaaccaccgctggtagcggtggtttttttgtttgcaagcagcagattacgcgcagaaaaaaaggatctcaagaagatcctttgatcttttctacggggtctgacgctcagtggaacgaaaactcacgttaagggattttggtcatgagattatcaaaaaggatcttcacctagatccttttaaattaaaaatgaagttttaaatcaatctaaagtatatatgagtaaacttggtctgacagttaccaatgcttaatcagtgaggcacctatctcagcgatctgtctatttcgttcatccatagttgcctgactccccgtcgtgtagataactacgatacgggagggcttaccatctggccccagtgctgcaatgataccgcgagacccacgctcaccggctccagatttatcagcaataaaccagccagccggaagggccgagcgcagaagtggtcctgcaactttatccgcctccatccagtctattaattgttgccgggaagctagagtaagtagttcgccagttaatagtttgcgcaacgttgttgccattgctacaggcatcgtggtgtcacgctcgtcgtttggtatggcttcattcagctccggttcccaacgatcaaggcgagttacatgatcccccatgttgtgcaaaaaagcggttagctccttcggtcctccgatcgttgtcagaagtaagttggccgcagtgttatcactcatggttatggcagcactgcataattctcttactgtcatgccatccgtaagatgcttttctgtgactggtgagtactcaaccaagtcattctgagaatagtgtatgcggcgaccgagttgctcttgcccggcgtcaatacgggataataccgcgccacatagcagaactttaaaagtgctcatcattggaaaacgttcttcggggcgaaaactctcaaggatcttaccgctgttgagatccagttcgatgtaacccactcgtgcacccaactgatcttcagcatcttttactttcaccagcgtttctgggtgagcaaaaacaggaaggcaaaatgccgcaaaaaagggaataagggcgacacggaaatgttgaatactcatactcttcctttttcaatattattgaagcatttatcagggttattgtctcatgagcggatacatatttgaatgtatttagaaaaataaacaaataggggttccgcgcacatttccccgaaaagtgccacctgacgtcgacggatcgggagatctcccgatcccctatggtgcactctcagtacaatctgctctgatgccgcatagttaagccagtatctgctccctgcttgtgtgttggaggtcgctgagtagtgcgcgagcaaaatttaagctacaacaaggcaaggcttgaccgacaattgcatgaagaatctgcttagggttaggcgttttgcgctgcttcgcgatgt

SEQ ID NO: 75 - DNA, 8127 bp, Artificial Sequence
  pRRL dual
ggtctctctggttagaccagatctgagcctgggagctctctggctaactagggaacccactgcttaagcctcaataaagcttgccttgagtgcttcaagtagtgtgtgcccgtctgttgtgtgactctggtaactagagatccctcagacccttttagtcagtgtggaaaatctctagcagtagtagttcatgtcatcttattattcagtatttataacttgcaaagaaatgaatatcagagagtgagaggaacttgtttattgcagcttataatggttacaaataaagcaatagcatcacaaatttcacaaataaagcatttttttcactgcattctagttgtggtttgtccaaactcatcaatgtatcttatcatgtctggctctagctatcccgcccctaactccgcccatcccgcccctaactccgcccagttccgcccattctccgccccatggctgactaattttttttatttatgcagaggccgaggccgcctcggcctctgagctattccagaagtagtgaggaggcttttttggaggcctagggacgtacccaattcgccctatagtgagtcgtattacgcgcgctcactggccgtcgttttacaacgtcgtgactgggaaaaccctggcgttacccaacttaatcgccttgcagcacatccccctttcgccagctggcgtaatagcgaagaggcccgcaccgatcgcccttcccaacagttgcgcagcctgaatggcgaatggcgcgacgcgccctgtagcggcgcattaagcgcggcgggtgtggtggttacgcgcagcgtgaccgctacacttgccagcgccctagcgcccgctcctttcgctttcttcccttcctttctcgccacgttcgccggctttccccgtcaagctctaaatcgggggctccctttagggttccgatttagtgctttacggcacctcgaccccaaaaaacttgattagggtgatggttcacgtagtgggccatcgccctgatagacggtttttcgccctttgacgttggagtccacgttctttaatagtggactcttgttccaaactggaacaacactcaaccctatctcggtctattcttttgatttataagggattttgccgatttcggcctattggttaaaaaatgagctgatttaacaaaaatttaacgcgaattttaacaaaatattaacgtttacaatttcccaggtggcacttttcggggaaatgtgcgcggaacccctatttgtttatttttctaaatacattcaaatatgtatccgctcatgagacaataaccctgataaatgcttcaataatattgaaaaaggaagagtatgagtattcaacatttccgtgtcgcccttattcccttttttgcggcattttgccttcctgtttttgctcacccagaaacgctggtgaaagtaaaagatgctgaagatcagttgggtgcacgagtgggttacatcgaactggatctcaacagcggtaagatccttgagagttttcgccccgaagaacgttttccaatgatgagcacttttaaagttctgctatgtggcgcggtattatcccgtattgacgccgggcaagagcaactcggtcgccgcatacactattctcagaatgacttggttgagtactcaccagtcacagaaaagcatcttacggatggcatgacagtaagagaattatgcagtgctgccataaccatgagtgataacactgcggccaacttacttctgacaacgatcggaggaccgaaggagctaaccgcttttttgcacaacatgggggatcatgtaactcgccttgatcgttgggaaccggagctgaatgaagccataccaaacgacgagcgtgacaccacgatgcctgtagcaatggcaacaacgttgcgcaaactattaactggcgaactacttactctagcttcccggcaacaattaatagactggatggaggcggataaagttgcaggaccacttctgcgctcggcccttccggctggctggtttattgctgataaatctggagccggtgagcgtgggtctcgcggtatcattgcagcactggggccagatggtaagccctcccgtatcgtagttatctacacgacggggagtcaggcaactatggatgaacgaaatagacagatcgctgagataggtgcctcactgattaagcattggtaactgtcagaccaagtttactcatatatactttagattgatttaaaacttcatttttaatttaaaaggatctaggtgaagatcctttttgataatctcatgaccaaaatcccttaacgtgagttttcgttccactgagcgtcagaccccgtagaaaagatcaaaggatcttcttgagatcctttttttctgcgcgtaatctgctgcttgcaaacaaaaaaaccaccgctaccagcggtggtttgtttgccggatcaagagctaccaactctttttccgaaggtaactggcttcagcagagcgcagataccaaatactgtccttctagtgtagccgtagttaggccaccacttcaagaactctgtagcaccgcctacatacctcgctctgctaatcctgttaccagtggctgctgccagtggcgataagtcgtgtcttaccgggttggactcaagacgatagttaccggataaggcgcagcggtcgggctgaacggggggttcgtgcacacagcccagcttggagcgaacgacctacaccgaactgagatacctacagcgtgagctatgagaaagcgccacgcttcccgaagggagaaaggcggacaggtatccggtaagcggcagggtcggaacaggagagcgcacgagggagcttccagggggaaacgcctggtatctttatagtcctgtcgggtttcgccacctctgacttgagcgtcgatttttgtgatgctcgtcaggggggcggagcctatggaaaaacgccagcaacgcggcctttttacggttcctggccttttgctggccttttgctcacatgttctttcctgcgttatcccctgattctgtggataaccgtattaccgcctttgagtgagctgataccgctcgccgcagccgaacgaccgagcgcagcgagtcagtgagcgaggaagcggaagagcgcccaatacgcaaaccgcctctccccgcgcgttggccgattcattaatgcagctggcacgacaggtttcccgactggaaagcgggcagtgagcgcaacgcaattaatgtgagttagctcactcattaggcaccccaggctttacactttatgcttccggctcgtatgttgtgtggaattgtgagcggataacaatttcacacaggaaacagctatgaccatgattacgtgccgcaagcttaatgtagtcttatgcaatactcttgtagtcttgcaacatggtaacgatgagttagcaacatgccttacaaggagagaaaaagcaccgtgcatgccgattggtggaagtaaggtggtacgatcgtgccttattaggaaggcaacagacgggtctgacatggattggacgaaccactgaattgccgcattgcagagatattgtatttaagtgcctagctcgatacaataaacgggtctctctggttagaccagatctgagcctgggagctctctggctaactagggaacccactgcttaagcctcaataaagcttgccttgagtgcttcaagtagtgtgtgcccgtctgttgtgtgactctggtaactagagatccctcagacccttttagtcagtgtggaaaatctctagcagtggcgcccgaacagggacctgaaagcgaaagggaaaccagagctctctcgacgcaggactcggcttgctgaagcgcgcacggcaagaggcgaggggcggcgactggtgagtacgccaaaaattttgactagcggaggctagaaggagagagatgggtgcgagagcgtcagcaagtattaagcgggggagaattagatcgcgatgggaaaaaattcggttaaggccagggggaaagaaaaaatataaattaaaacatatagtatgggcaagcagggagctagaacgattcgcagttaatcctggcctgttagaaacatcagaaggctgtagacaaatactgggacagctacaaccatcccttcagacaggatcagaagaacttagatcattatataatacagtagcaaccctctattgtgtgcatcaaaggatagagataaaagacaccaaggaagctttagacaagatagaggaagagcaaaacaaaagtaagaccaccgcacagcaagcggccggccgctgatcttcagacctggaggaggagatatgagggacaattggagaagtgaattatataaatataaagtagtaaaaattgaaccattaggagtagcacccaccaaggcaaagagaagagtggtgcagagagaaaaaagagcagtgggaataggagctttgttccttgggttcttgggagcagcaggaagcactatgggcgcagcgtcaatgacgctgacggtacaggccagacaattattgtctggtatagtgcagcagcagaacaatttgctgagggctattgaggcgcaacagcatctgttgcaactcacagtctggggcatcaagcagctccaggcaagaatcctggctgtggaaagatacctaaaggatcaacagctcctggggatttggggttgctctggaaaactcatttgcaccactgctgtgccttggaatgctagttggagtaataaatctctggaacagatttggaatcacacgacctggatggagtgggacagagaaattaacaattacacaagcttaatacactccttaattgaagaatcgcaaaaccagcaagaaaagaatgaacaagaattattggaattagataaatgggcaagtttgtggaattggtttaacataacaaattggctgtggtatataaaattattcataatgatagtaggaggcttggtaggtttaagaatagtttttgctgtactttctatagtgaatagagttaggcagggatattcaccattatcgtttcagacccacctcccaaccccgaggggacccgacaggcccgaaggaatagaagaagaaggtggagagagagacagagacagatccattcgattagtgaacggatcggcactgcgtgcgccaattctgcagacaaatggcagtattcatccacaattttaaaagaaaaggggggattggggggtacagtgcaggggaaagaatagtagacataatagcaacagacatacaaactaaagaattacaaaaacaaattacaaaaattcaaaattttcgggtttattacagggaactaaaggatctgcgatcgctccggtgcccgtcagtgggcagagcgcacatcgcccacagtccccgagaagttggggggaggggtcggcaattgaacgggtgcctagagaaggtggcgcggggtaaactgggaaagtgatgtcgtgtactggctccgcctttttcccgagggtgggggagaaccgtatataagtgcagtagtcgccgtgaacgttctttttcgcaacgggtttgccgccagaacacagctgaagcttcgaggggctcgcatctctccttcacgcgcccgccgccctacctgaggccgccatccacgccggttgagtcgcgttctgccgcctcccgcctgtggtgcctcctgaactgcgtccgccgtctaggtaagtttaaagctcaggtcgagaccgggcctttgtccggcgctcccttggagcctacctagactcagccggctctccacgctttgcctgaccctgcttgctcaactctacgtctttgtttcgttttctgttctgcgccgttacagatccaagctgtgaccggcgcctacgatatcgccaccatggccagctccgaggatgtcatcaaagagtttatgagatttaaggtcaagatggagggaagcgtcaacggacacgagttcgagattgagggagaaggagaaggccggccttacgagggcacacaaaccgctaagctcaaggtcacaaaaggaggacccctccccttctcctgggatattctgagccctcagttccagtacggaagcaaagcctatgttaaacaccctgccgacatccctgactatctgaagctctccttccctgaaggcttcaagtgggagagattcatgaacttcgaggacggaggcgtggtgacagtcacacaagatagcaccctccaggacggagagtttatttataaggtgaaactcagaggaaccaacttcccctccgatggccctgtcatgcaaaaaaaaacaatgggatgggaagcctccaccgagagaatgtatcctgaggatggcgctctgaaaggcgaaattaaaatgagactgaaactcaaagacggaggacactacgatgccgaggtcaaaacaacctacaaggccaagaaacaagtgcagctgcctggcgcctacatgactgatattaaactcgacattatcagccataatggggactacaccatcgtggaacaatatgagagagctgagggcagacatagcacaggcgctggaggctccggggcaacgaatttcagtctgcttaaacaagcaggagatgttgaagagaatcctggtcccatggtgtctaagggcgaagagctctttactggcgtggtgcccatcctggttgaattggacggagatgttaacggacacaaatttagcgtatctggagagggcgaaggtaagtaatcggttcaagtgattctcctgcctcagcctcccaagtagctgggattagaggtccccaccaccatgcctggctaattttttgtactttcagtagaaatggggttttgccatgttggccaggctgttctcgaactcctgagctcaggtgatccaactgtctcggcctcccaaagtgctgggattacaggcgtgagccactgtgcctagcctgagccaccacgccggcctaatttttaaattttttgtagagacagggtctcattatgttgcccagggtggtgtcaagctccaggtctcaagtgatccccctacctccgcctcccaaagttgtgggattgtaggcatgagccactgcaagaaaaccttaactgcagcctaataattgttttctttgggataacttttaaagtacattaaaagactatcaacttaatttctgatcatattttgttgaataaaataagtaaaatgtcttgtgaaacaaaatgctttttaacatccatataaagctatctatatatagctatctatgtctggcgcgccgagcgaattccgtttaagaccaatgacttacaaggcagctgtagatcttagccactttttaaaagaaaaggggggactggaagggctaattcactcccaacgaagacaagatatgatcaaagcttggccattgcatacgttgtatccatatcataatatgtacatttatattggctcatgtccaacattaccgccatgttgacattgattattgactagttattaatagtaatcaattacggggtcattagttcatagcccatatatggagttccgcgttacataacttacggtaaatggcccgcctggctgaccgcccaacgacccccgcccattgacgtcaataatgacgtatgttcccatagtaacgccaatagggactttccattgacgtcaatgggtggagtatttacggtaaactgcccacttggcagtacatcaagtgtatcatatgccaagtacgccccctattgacgtcaatgacggtaaatggcccgcctggcattatgcccagtacatgaccttatgggactttcctacttggcagtacatctacgtattagtcatcgctattaccatggtgatgcggttttggcagtacatcaatgggcgtggatagcggtttgactcacggggatttccaagtctccaccccattgacgtcaatgggagtttgttttggcaccaaaatcaacgggactttccaaaatgtcgtaacaactccgccccattgacgcaaatgggcggtaggcgtgtacggtgggaggtctatataagcagagctcgtttagtgaaccgg

SEQ ID NO: 76 - DNA, 8005 bp, Artificial Sequence
  psMCP-GAG
ttaagccagtatctgctccctgcttgtgtgttggaggtcgctgagtagtgcgcgagcaaaatttaagctacaacaaggcaaggcttgaccgacaattgcatgaagaatctgcttagggttaggcgttttgcgctgcttcgcgatgtacgggccagatatacgcgttgacattgattattgactagttattaatagtaatcaattacggggtcattagttcatagcccatatatggagttccgcgttacataacttacggtaaatggcccgcctggctgaccgcccaacgacccccgcccattgacgtcaataatgacgtatgttcccatagtaacgccaatagggactttccattgacgtcaatgggtggagtatttacggtaaactgcccacttggcagtacatcaagtgtatcatatgccaagtacgccccctattgacgtcaatgacggtaaatggcccgcctggcattatgcccagtacatgaccttatgggactttcctacttggcagtacatctacgtattagtcatcgctattaccatggtgatgcggttttggcagtacatcaatgggcgtggatagcggtttgactcacggggatttccaagtctccaccccattgacgtcaatgggagtttgttttggcaccaaaatcaacgggactttccaaaatgtcgtaacaactccgccccattgacgcaaatgggcggtaggcgtgtacggtgggaggtctatataagcagagctctctggctaactagagaacccactgcttactggcttatcgaaattaatacgactcactatagggagacccaagcttggtaccgagctcggatccactagtaacggccgccagtgtgctggaattcaccggtgcccgccaccatggcctctaattttactcaatttgtgcttgtcgataatggggggacgggagatgtgaccgttgcccctagcaatttcgcaaatggcgttgcagaatggatctctagcaacagcagaagccaagcgtacaaagtaacgtgttccgttcgccaaagctccgcccaaaaacggaagtatacaataaaggttgaggtgccgaaagtagccactcaaacagttggtggggtagaattgcccgtagcggcatggcggtcatatctcaatatggaactcactatcccaatcttcgccacgaatagcgattgtgagctgatagttaaggctatgcaaggtcttctcaaagatggaaaccctattccatctgctatcgccgccaacagcgggatatacagccagaactatccgattgtgcagtccggactcagatctcgagctcaagcttcgaattctgcagtcgacggtaccgcgggcccgggatccatggactcgggccgggacttcctgaccctgcacggcctacaggatgatgaggatctacaggcgctgctgaagggcagccagctcctgaaggtgaagtccagctcatggaggagagagcgcttctacaagttgcaggaggactgcaagaccatctggcaggagtcccgcaaggtcatgcggaccccggagtcccagctgttctccatcgaggacattcaggaggtgcgaatggggcaccgcacggagggtctggagaagttcgcccgtgatgtgcccgaggaccgctgcttctccattgtcttcaaggaccagcgcaatacactagacctcatcgccccatcgccagctgatgcccagcactgggtgctggggctgcacaagatcatccaccactcaggctccatggaccagcgtcagaagctacagcactggattcactcctgcttgcgaaaagctgacaaaaacaaggacaacaagatgagcttcaaggagctgcagaacttcctgaaggagctcaacatccagcctcgagccgaattcaccctggccgccagggccagcgtgctgagcggcggcgagctggacaggtgggagaagatcaggctgaggcccggcggcaagaagaagtataagctgaagcacatcgtgtgggccagcagggagctggagaggttcgccgtgaaccccggcctgctggagaccagcgagggctgcaggcagatcctgggccagctgcagcccagcctgcagaccggcagcgaggagctgaggagcctgtacaacaccgtggccaccctgtactgcgtgcaccagaggatcgagatcaaggacaccaaggaggccctggacaagatcgaggaggagcagaacaagtccaagaagaaggcccagcaggccgccgccgacaccggccacagcagccaggtgagccagaactaccccatcgtgcagaacatccagggccagatggtgcaccaggccatcagccccaggaccctgaacgcctgggtgaaggtggtggaggagaaggccttcagccccgaggtgatccccatgttcagcgccctgagcgagggagccaccccccaggacctgaacaccatgctgaacaccgtgggcggccaccaggccgccatgcagatgctgaaggagaccatcaacgaggaggccgccgagtgggacagggtgcaccccgtgcacgccggccccatcgcccccggccagatgagggagccccgcggcagcgacatcgccggcaccaccagcaccctgcaggagcagatcggctggatgaccaacaacccccccatccccgtgggcgaaatctacaagaggtggatcatcctgggcctgaacaagatcgtgaggatgtacagccccaccagcatcctggatatcaggcagggccccaaagagcccttcagggactacgtggacaggttctacaagaccctgcgcgccgagcaggccagccaggaggtgaagaactggatgaccgagaccctgctggtgcagaacgccaaccccgactgcaagaccatcctgaaggccctgggacccgccgccaccctggaggagatgatgaccgcctgccagggcgtgggcggccccggccacaaggccagggtgctggccgaggccatgagccaggtgaccaacaccgccaccatcatgatgcagaggggcaacttcaggaaccagaggaagatggtgaagtgcttcaactgcggcaaggagggccacaccgccaggaactgccgcgcccccaggaagaagggctgctggaagtgcggcaaggagggccaccagatgaaggactgcaccgagaggcaggctaattttttagggaagatctggccttcctacaagggaaggccagggaattttcttcagagcagaccagagccaacagccccaccatttcttcagagcagaccagagccaacagccccaccagaagagagcttcaggtctggggtagagacaacaactccccctcagaagcaggagccgatagacaaggaactgtatcctttaacttccctcagatcactctttggcaacgacccctcgtcacaataactgccgcggccgctcgagcatgcatctagagggccctattctatagtgtcacctaaatgctagagctcgctgatcagcctcgactgtgccttctagttgccagccatctgttgtttgcccctcccccgtgccttccttgaccctggaaggtgccactcccactgtcctttcctaataaaatgaggaaattgcatcgcattgtctgagtaggtgtcattctattctggggggtggggtggggcaggacagcaagggggaggattgggaagacaatagcaggcatgctggggatgcggtgggctctatggcttctgaggcggaaagaaccagctggggctctagggggtatccccacgcgccctgtagcggcgcattaagcgcggcgggtgtggtggttacgcgcagcgtgaccgctacacttgccagcgccctagcgcccgctcctttcgctttcttcccttcctttctcgccacgttcgccggctttccccgtcaagctctaaatcgggggctccctttagggttccgatttagtgctttacggcacctcgaccccaaaaaacttgattagggtgatggttcacgtagtgggccatcgccctgatagacggtttttcgccctttgacgttggagtccacgttctttaatagtggactcttgttccaaactggaacaacactcaaccctatctcggtctattcttttgatttataagggattttgccgatttcggcctattggttaaaaaatgagctgatttaacaaaaatttaacgcgaattaattctgtggaatgtgtgtcagttagggtgtggaaagtccccaggctccccagcaggcagaagtatgcaaagcatgcatctcaattagtcagcaaccaggtgtggaaagtccccaggctccccagcaggcagaagtatgcaaagcatgcatctcaattagtcagcaaccatagtcccgcccctaactccgcccatcccgcccctaactccgcccagttccgcccattctccgccccatggctgactaattttttttatttatgcagaggccgaggccgcctctgcctctgagctattccagaagtagtgaggaggcttttttggaggcctaggcttttgcaaaaagctcccgggagcttgtatatccattttcggatctgatcaagagacaggatgaggatcgtttcgcatgattgaacaagatggattgcacgcaggttctccggccgcttgggtggagaggctattcggctatgactgggcacaacagacaatcggctgctctgatgccgccgtgttccggctgtcagcgcaggggcgcccggttctttttgtcaagaccgacctgtccggtgccctgaatgaactgcaggacgaggcagcgcggctatcgtggctggccacgacgggcgttccttgcgcagctgtgctcgacgttgtcactgaagcgggaagggactggctgctattgggcgaagtgccggggcaggatctcctgtcatctcaccttgctcctgccgagaaagtatccatcatggctgatgcaatgcggcggctgcatacgcttgatccggctacctgcccattcgaccaccaagcgaaacatcgcatcgagcgagcacgtactcggatggaagccggtcttgtcgatcaggatgatctggacgaagagcatcaggggctcgcgccagccgaactgttcgccaggctcaaggcgcgcatgcccgacggcgaggatctcgtcgtgacccatggcgatgcctgcttgccgaatatcatggtggaaaatggccgcttttctggattcatcgactgtggccggctgggtgtggcggaccgctatcaggacatagcgttggctacccgtgatattgctgaagagcttggcggcgaatgggctgaccgcttcctcgtgctttacggtatcgccgctcccgattcgcagcgcatcgccttctatcgccttcttgacgagttcttctgagcgggactctggggttcgaaatgaccgaccaagcgacgcccaacctgccatcacgagatttcgattccaccgccgccttctatgaaaggttgggcttcggaatcgttttccgggacgccggctggatgatcctccagcgcggggatctcatgctggagttcttcgcccaccccaacttgtttattgcagcttataatggttacaaataaagcaatagcatcacaaatttcacaaataaagcatttttttcactgcattctagttgtggtttgtccaaactcatcaatgtatcttatcatgtctgtataccgtcgacctctagctagagcttggcgtaatcatggtcatagctgtttcctgtgtgaaattgttatccgctcacaattccacacaacatacgagccggaagcataaagtgtaaagcctggggtgcctaatgagtgagctaactcacattaattgcgttgcgctcactgcccgctttccagtcgggaaacctgtcgtgccagctgcattaatgaatcggccaacgcgcggggagaggcggtttgcgtattgggcgctcttccgcttcctcgctcactgactcgctgcgctcggtcgttcggctgcggcgagcggtatcagctcactcaaaggcggtaatacggttatccacagaatcaggggataacgcaggaaagaacatgtgagcaaaaggccagcaaaaggccaggaaccgtaaaaaggccgcgttgctggcgtttttccataggctccgcccccctgacgagcatcacaaaaatcgacgctcaagtcagaggtggcgaaacccgacaggactataaagataccaggcgtttccccctggaagctccctcgtgcgctctcctgttccgaccctgccgcttaccggatacctgtccgcctttctcccttcgggaagcgtggcgctttctcatagctcacgctgtaggtatctcagttcggtgtaggtcgttcgctccaagctgggctgtgtgcacgaaccccccgttcagcccgaccgctgcgccttatccggtaactatcgtcttgagtccaacccggtaagacacgacttatcgccactggcagcagccactggtaacaggattagcagagcgaggtatgtaggcggtgctacagagttcttgaagtggtggcctaactacggctacactagaagaacagtatttggtatctgcgctctgctgaagccagttaccttcggaaaaagagttggtagctcttgatccggcaaacaaaccaccgctggtagcggtttttttgtttgcaagcagcagattacgcgcagaaaaaaaggatctcaagaagatcctttgatcttttctacggggtctgacgctcagtggaacgaaaactcacgttaagggattttggtcatgagattatcaaaaaggatcttcacctagatccttttaaattaaaaatgaagttttaaatcaatctaaagtatatatgagtaaacttggtctgacagttaccaatgcttaatcagtgaggcacctatctcagcgatctgtctatttcgttcatccatagttgcctgactccccgtcgtgtagataactacgatacgggagggcttaccatctggccccagtgctgcaatgataccgcgagacccacgctcaccggctccagatttatcagcaataaaccagccagccggaagggccgagcgcagaagtggtcctgcaactttatccgcctccatccagtctattaattgttgccgggaagctagagtaagtagttcgccagttaatagtttgcgcaacgttgttgccattgctacaggcatcgtggtgtcacgctcgtcgtttggtatggcttcattcagctccggttcccaacgatcaaggcgagttacatgatcccccatgttgtgcaaaaaagcggttagctccttcggtcctccgatcgttgtcagaagtaagttggccgcagtgttatcactcatggttatggcagcactgcataattctcttactgtcatgccatccgtaagatgcttttctgtgactggtgagtactcaaccaagtcattctgagaatagtgtatgcggcgaccgagttgctcttgcccggcgtcaatacgggataataccgcgccacatagcagaactttaaaagtgctcatcattggaaaacgttcttcggggcgaaaactctcaaggatcttaccgctgttgagatccagttcgatgtaacccactcgtgcacccaactgatcttcagcatcttttactttcaccagcgtttctgggtgagcaaaaacaggaaggcaaaatgccgcaaaaaagggaataagggcgacacggaaatgttgaatactcatactcttcctttttcaatattattgaagcatttatcagggttattgtctcatgagcggatacatatttgaatgtatttagaaaaataaacaaataggggttccgcgcacatttccccgaaaagtgccacctgacgtcgacggatcgggagatctcccgatcccctatggtgcactctcagtacaatctgctctgatgccgcatag

SEQ ID NO: 77 - DNA, 10711 bp, Artificial Sequence
  psMCP-GAGPOL
gacggatcgggagatctcccgatcccctatggtgcactctcagtacaatctgctctgatgccgcatagttaagccagtatctgctccctgcttgtgtgttggaggtcgctgagtagtgcgcgagcaaaatttaagctacaacaaggcaaggcttgaccgacaattgcatgaagaatctgcttagggttaggcgttttgcgctgcttcgcgatgtacgggccagatatacgcgttgacattgattattgactagttattaatagtaatcaattacggggtcattagttcatagcccatatatggagttccgcgttacataacttacggtaaatggcccgcctggctgaccgcccaacgacccccgcccattgacgtcaataatgacgtatgttcccatagtaacgccaatagggactttccattgacgtcaatgggtggagtatttacggtaaactgcccacttggcagtacatcaagtgtatcatatgccaagtacgccccctattgacgtcaatgacggtaaatggcccgcctggcattatgcccagtacatgaccttatgggactttcctacttggcagtacatctacgtattagtcatcgctattaccatggtgatgcggttttggcagtacatcaatgggcgtggatagcggtttgactcacggggatttccaagtctccaccccattgacgtcaatgggagtttgttttggcaccaaaatcaacgggactttccaaaatgtcgtaacaactccgccccattgacgcaaatgggcggtaggcgtgtacggtgggaggtctatataagcagagctggtttagtgaaccgtcagatccgctagcgctaccggtcgccaccatggcctctaattttactcaatttgtgcttgtcgataatggggggacgggagatgtgaccgttgcccctagcaatttcgcaaatggcgttgcagaatggatctctagcaacagcagaagccaagcgtacaaagtaacgtgttccgttcgccaaagctccgcccaaaaacggaagtatacaataaaggttgaggtgccgaaagtagccactcaaacagttggtggggtagaattgcccgtagcggcatggcggtcatatctcaatatggaactcactatcccaatcttcgccacgaatagcgattgtgagctgatagttaaggctatgcaaggtcttctcaaagatggaaaccctattccatctgctatcgccgccaacagcgggatatacagccagaactatccgattgtgcagtccggactcagatctcgagctcaagcttcgaattctgcagtcgacggtaccgcgggcccgggatccatggactcgggccgggacttcctgaccctgcacggcctacaggatgatgaggatctacaggcgctgctgaagggcagccagctcctgaaggtgaagtccagctcatggaggagagagcgcttctacaagttgcaggaggactgcaagaccatctggcaggagtcccgcaaggtcatgcggaccccggagtcccagctgttctccatcgaggacattcaggaggtgcgaatggggcaccgcacggagggtctggagaagttcgcccgtgatgtgcccgaggaccgctgcttctccattgtcttcaaggaccagcgcaatacactagacctcatcgccccatcgccagctgatgcccagcactgggtgctggggctgcacaagatcatccaccactcaggctccatggaccagcgtcagaagctacagcactggattcactcctgcttgcgaaaagctgacaaaaacaaggacaacaagatgagcttcaaggagctgcagaacttcctgaaggagctcaacatccagcctcgagccgaattcaccctggccgccagggccagcgtgctgagcggcggcgagctggacaggtgggagaagatcaggctgaggcccggcggcaagaagaagtataagctgaagcacatcgtgtgggccagcagggagctggagaggttcgccgtgaaccccggcctgctggagaccagcgagggctgcaggcagatcctgggccagctgcagcccagcctgcagaccggcagcgaggagctgaggagcctgtacaacaccgtggccaccctgtactgcgtgcaccagaggatcgagatcaaggacaccaaggaggccctggacaagatcgaggaggagcagaacaagtccaagaagaaggcccagcaggccgccgccgacaccggccacagcagccaggtgagccagaactaccccatcgtgcagaacatccagggccagatggtgcaccaggccatcagccccaggaccctgaacgcctgggtgaaggtggtggaggagaaggccttcagccccgaggtgatccccatgttcagcgccctgagcgagggagccaccccccaggacctgaacaccatgctgaacaccgtgggcggccaccaggccgccatgcagatgctgaaggagaccatcaacgaggaggccgccgagtgggacagggtgcaccccgtgcacgccggccccatcgcccccggccagatgagggagccccgcggcagcgacatcgccggcaccaccagcaccctgcaggagcagatcggctggatgaccaacaacccccccatccccgtgggcgaaatctacaagaggtggatcatcctgggcctgaacaagatcgtgaggatgtacagccccaccagcatcctggatatcaggcagggccccaaagagcccttcagggactacgtggacaggttctacaagaccctgcgcgccgagcaggccagccaggaggtgaagaactggatgaccgagaccctgctggtgcagaacgccaaccccgactgcaagaccatcctgaaggccctgggacccgccgccaccctggaggagatgatgaccgcctgccagggcgtgggcggccccggccacaaggccagggtgctggccgaggccatgagccaggtgaccaacaccgccaccatcatgatgcagaggggcaacttcaggaaccagaggaagatggtgaagtgcttcaactgcggcaaggagggccacaccgccaggaactgccgcgcccccaggaagaagggctgctggaagtgcggcaaggagggccaccagatgaaggactgcaccgagaggcaggctaattttttagggaagatctggccttcctacaagggaaggccagggaattttcttcagagcagaccagagccaacagccccaccatttcttcagagcagaccagagccaacagccccaccagaagagagcttcaggtctggggtagagacaacaactccccctcagaagcaggagccgatagacaaggaactgtatcctttaacttccctcagatcactctttggcaacgacccctcgtcacaataaagatcggtggccagctgaaggaggccctgctggacaccggcgccgacgacaccgtgctggaggagatgagcctgcccggcaggtggaagcccaagatgatcggcggcatcggcggcttcatcaaggtgaggcagtacgaccagatcctgatcgagatctgcggccacaaggccatcggcaccgtgctggtgggacctacacctgtgaacatcatcggcaggaacctgctgacccagatcggctgcaccctgaacttccccatcagccccatcgagaccgtgcccgtgaagctgaagcccggcatggacggccctaaggtgaagcagtggcccctgaccgaggagaagatcaaggccctggtggagatctgcaccgagatggagaaggagggcaagatcagcaagatcggccccgagaacccctacaacacccccgtgttcgccatcaagaagaaggacagcaccaagtggaggaagctggtggacttcagggagctgaacaagaggacccaggacttctgggaggtgcagctgggcatcccccaccccgccggcctgaagaagaagaagagcgtgaccgtgctggacgtgggcgacgcctacttcagcgtgcccctggacgaggacttcaggaagtataccgccttcaccatccccagcatcaacaacgagacccccggcatccgctaccagtacaacgtgctgccccagggctggaagggcagccccgccatcttccagagcagcatgacaaagatcctggagcccttcaagaagcagaaccccgacatcgtgatctatcagtacatggacgacctgtacgtgggcagcgacctggagatcggccagcacaggaccaagatcgaggagctgaggcagcacctgctgaggtggggcctgaccacccccgacaagaagcaccagaaggagcccccattcctgtggatgggctacgagctgcaccccgacaagtggaccgtgcagcccatcgtgctgcccgagaaggacagctggaccgtgaacgacattcagaagctggtgggcaagctgaactgggccagccagatctaccctggcatcaaggtgaggcagctgtgcaagctgctgaggggcacaaaggctctgaccgaggtgatccccctgaccgaggaggccgagctggagctggccgagaacagggagatcctgaaggagcccgtgcacggcgtgtactacgaccccagcaaggacctgatcgccgagatccagaagcagggccagggccagtggacctaccagatctaccaggagcccttcaagaacctgaagaccggcaagtacgcccgcatgcgcggcgcccacaccaacgacgtgaagcagctgaccgaggccgtgcagaagatcaccaccgagagcatcgtgatctggggcaagactcctaagttcaagctgcccatccagaaggagacctgggagacctggtggaccgagtactggcaggccacctggattcccgagtgggagttcgtgaacacccctcccctggtgaagctgtggtatcagctggagaaggagcccatcgtgggcgccgagaccttctacgtggacggcgccgccaacagggagaccaagctgggcaaggccggctacgtgaccaacaagggccgccagaaggtggtgcccctgaccaacaccaccaaccagaagaccgagctgcaggctatctacctggccctgcaggactcaggcctggaggtgaacatcgtgaccgacagccagtacgccctgggcatcatccaggcccagcccgacaagagcgagagcgagctggtgaaccagatcatcgagcagctgatcaagaaggagaaggtgtacctggcctgggtgcccgcccacaagggcatcggcggcaacgagcaggtggacaagctggtgagcgccggcatcaggaagatcctgttcctggacggcatcgacaaggcccaggacgagcacgagaagtaccacagcaactggagggctatggctagcgacttcaacctgcctcccgtggtggctaaggagatcgtggccagctgcgacaagtgccagctgaagggcgaggccatgcacggccaggtggactgcagccccggcatctggcagctggattgcacccacctggagggcaaggtgatcctggtggccgtgcacgtggcctccggctacatcgaggccgaggtgatccccgccgagaccggccaggagaccgcctacttcctgctgaagctggccggccgctggcccgtgaagaccatccacaccgacaacggcagcaacttcaccagcgccaccgtgaaggctgcctgctggtgggccggcatcaagcaggagttcggcatcccctacaacccccagtctcagggcgtggtggagagcatgaacaaggagctgaagaagatcatcggccaggtgagggaccaggccgagcacctgaagaccgccgtgcagatggccgtgttcatccacaacttcaagaggaagggcggcatcggcggctacagcgccggcgagaggatcgtggacatcatcgccaccgacatccagaccaaggagctgcagaagcagatcaccaagatccagaacttcagggtgtactacagggacagcaggaaccctctgtggaagggccccgccaagctgctgtggaagggcgagggcgccgtggtgatccaggacaacagcgacatcaaggtggtgcccaggaggaaggccaagatcatcagggactacggcaagcagatggccggcgacgactgcgtggcctccaggcaggacgaggactgataaggatccctcgagcatgcatctagagggccctattctatagtgtcacctaaatgctagagctcgctgatcagcctcgactgtgccttctagttgccagccatctgttgtttgcccctcccccgtgccttccttgaccctggaaggtgccactcccactgtcctttcctaataaaatgaggaaattgcatcgcattgtctgagtaggtgtcattctattctggggggtggggtggggcaggacagcaagggggaggattgggaagacaatagcaggcatgctggggatgcggtgggctctatggcttctgaggcggaaagaaccagctggggctctagggggtatccccacgcgccctgtagcggcgcattaagcgcggcgggtgtggtggttacgcgcagcgtgaccgctacacttgccagcgccctagcgcccgctcctttcgctttcttcccttcctttctcgccacgttcgccggctttccccgtcaagctctaatcgggggctccctttagggttccgatttagtgctttacggcacctcgaccccaaaaaacttgattagggtgatggttcacgtagtgggccatcgccctgatagacggtttttcgccctttgacgttggagtccacgttctttaatagtggactcttgttccaaactggaacaacactcaaccctatctcggtctattcttttgatttataagggattttgccgatttcggcctattggttaaaaaatgagctgatttaacaaaaatttaacgcgaattaattctgtggaatgtgtgtcagttagggtgtggaaagtccccaggctccccagcaggcagaagtatgcaaagcatgcatctcaattagtcagcaaccaggtgtggaaagtccccaggctccccagcaggcagaagtatgcaaagcatgcatctcaattagtcagcaaccatagtcccgcccctaactccgcccatcccgcccctaactccgcccagttccgcccattctccgccccatggctgactaattttttttatttatgcagaggccgaggccgcctctgcctctgagctattccagaagtagtgaggaggcttttttggaggcctaggcttttgcaaaaagctcccgggagcttgtatatccattttcggatctgatcaagagacaggatgaggatcgtttcgcatgattgaacaagatggattgcacgcaggttctccggccgcttgggtggagaggctattcggctatgactgggcacaacagacaatcggctgctctgatgccgccgtgttccggctgtcagcgcaggggcgcccggttctttttgtcaagaccgacctgtccggtgccctgaatgaactgcaggacgaggcagcgcggctatcgtggctggccacgacgggcgttccttgcgcagctgtgctcgacgttgtcactgaagcgggaagggactggctgctattgggcgaagtgccggggcaggatctcctgtcatctcaccttgctcctgccgagaaagtatccatcatggctgatgcaatgcggcggctgcatacgcttgatccggctacctgcccattcgaccaccaagcgaaacatcgcatcgagcgagcacgtactcggatggaagccggtcttgtcgatcaggatgatctggacgaagagcatcaggggctcgcgccagccgaactgttcgccaggctcaaggcgcgcatgcccgacggcgaggatctcgtcgtgacccatggcgatgcctgcttgccgaatatcatggtggaaaatggccgcttttctggattcatcgactgtggccggctgggtgtggcggaccgctatcaggacatagcgttggctacccgtgatattgctgaagagcttggcggcgaatgggctgaccgcttcctcgtgctttacggtatcgccgctcccgattcgcagcgcatcgccttctatcgccttcttgacgagttcttctgagcgggactctggggttcgaaatgaccgaccaagcgacgcccaacctgccatcacgagatttcgattccaccgccgccttctatgaaaggttgggcttcggaatcgttttccgggacgccggctggatgatcctccagcgcggggatctcatgctggagttcttcgcccaccccaacttgtttattgcagcttataatggttacaaataaagcaatagcatcacaaatttcacaaataaagcatttttttcactgcattctagttgtggtttgtccaaactcatcaatgtatcttatcatgtctgtataccgtcgacctctagctagagcttggcgtaatcatggtcatagctgtttcctgtgtgaaattgttatccgctcacaattccacacaacatacgagccggaagcataaagtgtaaagcctggggtgcctaatgagtgagctaactcacattaattgcgttgcgctcactgcccgctttccagtcgggaaacctgtcgtgccagctgcattaatgaatcggccaacgcgcggggagaggcggtttgcgtattgggcgctcttccgcttcctcgctcactgactcgctgcgctcggtcgttcggctgcggcgagcggtatcagctcactcaaaggcggtaatacggttatccacagaatcaggggataacgcaggaaagaacatgtgagcaaaaggccagcaaaaggccaggaaccgtaaaaaggccgcgttgctggcgtttttccataggctccgcccccctgacgagcatcacaaaaatcgacgctcaagtcagaggtggcgaaacccgacaggactataaagataccaggcgtttccccctggaagctccctcgtgcgctctcctgttccgaccctgccgcttaccggatacctgtccgcctttctcccttcgggaagcgtggcgctttctcatagctcacgctgtaggtatctcagttcggtgtaggtcgttcgctccaagctgggctgtgtgcacgaaccccccgttcagcccgaccgctgcgccttatccggtaactatcgtcttgagtccaacccggtaagacacgacttatcgccactggcagcagccactggtaacaggattagcagagcgaggtatgtaggcggtgctacagagttcttgaagtggtggcctaactacggctacactagaagaacagtatttggtatctgcgctctgctgaagccagttaccttcggaaaaagagttggtagctcttgatccggcaaacaaaccaccgctggtagcggtggtttttttgtttgcaagcagcagattacgcgcagaaaaaaaggatctcaagaagatcctttgatcttttctacggggtctgacgctcagtggaacgaaaactcacgttaagggattttggtcatgagattatcaaaaaggatcttcacctagatccttttaaattaaaaatgaagttttaaatcaatctaaagtatatatgagtaaacttggtctgacagttaccaatgcttaatcagtgaggcacctatctcagcgatctgtctatttcgttcatccatagttgcctgactccccgtcgtgtagataactacgatacgggagggcttaccatctggccccagtgctgcaatgataccgcgagacccacgctcaccggctccagatttatcagcaataaaccagccagccggaagggccgagcgcagaagtggtcctgcaactttatccgcctccatccagtctattaattgttgccgggaagctagagtaagtagttcgccagttaatagtttgcgcaacgttgttgccattgctacaggcatcgtggtgtcacgctcgtcgtttggtatggcttcattcagctccggttcccaacgatcaaggcgagttacatgatcccccatgttgtgcaaaaaagcggttagctccttcggtcctccgatcgttgtcagaagtaagttggccgcagtgttatcactcatggttatggcagcactgcataattctcttactgtcatgccatccgtaagatgcttttctgtgactggtgagtactcaaccaagtcattctgagaatagtgtatgcggcgaccgagttgctcttgcccggcgtcaatacgggataataccgcgccacatagcagaactttaaaagtgctcatcattggaaaacgttcttcggggcgaaaactctcaaggatcttaccgctgttgagatccagttcgatgtaacccactcgtgcacccaactgatcttcagcatcttttactttcaccagcgtttctgggtgagcaaaaacaggaaggcaaaatgccgcaaaaaagggaataagggcgacacggaaatgttgaatactcatactcttcctttttcaatattattgaagcatttatcagggttattgtctcatgagcggatacatatttgaatgtatttagaaaaataaacaaataggggttccgcgcacatttccccgaaaagtgccacctgacgtc

SEQ ID NO: 78 - protein, 442 aa, Artificial Sequence
  Cas12f
MAPKKKRKVMIKVYRYEIVKPLDLDWKEFGTILRQLQQETRFALNKATQLAWEWMGFSSDYKDNHGEYPKSKDILGYTNVHGYAYHTIKTKAYRLNSGNLSQTIKRATDRFKAYQKEILRGDMSIPSYKRDIPLDLIKENISVNRMNHGDYIASLSLLSNPAKQEMNVKRKISVIIIVRGAGKTIMDRILSGEYQVSASQIIHDDRKNKWYLNISYDFEPQTRVLDLNKIMGIDLGVAVAVYMAFQHTPARYKLEGGEIENFRRQVESRRISMLRQGKYAGGARGGHGRDKRIKPIEQLRDKIANFRDTTNHRYSRYIVDMAIKEGCGTIQMEDLTNIRDIGSRFLQNWTYYDLQQKIIYKAEEAGIKVIKIDPQYTSQRCSECGNIDSGNRIGQAIFKCRACGYEANADYNAARNIAIPNIDKIIAESIKSGGSPKKKRKV